European Patent Specification EP 3 573 623 B1, published March 4, 2026. Title: Compositions and Methods for Inhibition of Factor XII Gene Expression. Applicant: ARROWHEAD PHARMACEUTICALS, INC. The sequence listing filed with the application follows.

SEQUENCE LISTING (1027 sequences)

SEQ ID NO: 1 - DNA, 2060 bp, Homo sapiens
  Coagulation factor XII (12), complete gene (NM_000505.3)
ctattgatctggactcctggataggcagctggaccaacggacggatgccatgagggctctgctgctcctggggttcctgctggtgagcttggagtcaacactttcgattccaccttgggaagcccccaaggagcataagtacaaagctgaagagcacacagtcgttctcactgtcaccggggagccctgccacttccccttccagtaccaccggcagctgtaccacaaatgtacccacaagggccggccaggccctcagccctggtgtgctaccacccccaactttgatcaggaccagcgatggggatactgtttggagcccaagaaagtgaaagaccactgcagcaaacacagcccctgccagaaaggagggacctgtgtgaacatgccaagcggcccccactgtctctgtccacaacacctcactggaaaccactgccagaaagagaagtgctttgagcctcagcttctccggtttttccacaagaatgagatatggtatagaactgagcaagcagctgtggccagatgccagtgcaagggtcctgatgcccactgccagcggctggccagccaggcctgccgcaccaacccgtgcctccatgggggtcgctgcctagaggtggagggccaccgcctgtgccactgcccggtgggctacaccggagccttctgcgacgtggacaccaaggcaagctgctatgatggccgcgggctcagctaccgcggcctggccaggaccacgctctcgggtgcgccctgtcagccgtgggcctcggaggccacctaccggaacgtgactgccgagcaagcgcggaactggggactgggcggccacgccttctgccggaacccggacaacgacatccgcccgtggtgcttcgtgctgaaccgcgaccggctgagctgggagtactgcgacctggcacagtgccagaccccaacccaggcggcgcctccgaccccggtgtcccctaggcttcatgtcccactcatgcccgcgcagccggcaccgccgaagcctcagcccacgacccggaccccgcctcagtcccagaccccgggagccttgccggcgaagcgggagcagccgccttccctgaccaggaacggcccactgagctgcgggcagcggctccgcaagagtctgtcttcgatgacccgcgtcgttggcgggctggtggcgctacgcggggcgcacccctacatcgccgcgctgtactggggccacagtttctgcgccggcagcctcatcgccccctgctgggtgctgacggccgctcactgcctgcaggaccggcccgcacccgaggatctgacggtggtgctcggccaggaacgccgtaaccacagctgtgagccgtgccagacgttggccgtgcgctcctaccgcttgcacgaggccttctcgcccgtcagctaccagcacgacctggctctgttgcgccttcaggaggatgcggacggcagctgcgcgctcctgtcgccttacgttcagccggtgtgcctgccaagcggcgccgcgcgaccctccgagaccacgctctgccaggtggccggctggggccaccagttcgagggggcggaggaatatgccagcttcctgcaggaggcgcaggtaccgttcctctccctggagcgctgctcagccccggacgtgcacggatcctccatcctccccggcatgctctgcgcagggttcctcgagggcggcaccgatgcgtgccagggtgattccggaggcccgctggtgtgtgaggaccaagctgcagagcgccggctcaccctgcaaggcatcatcagctggggatcgggctgtggtgaccgcaacaagccaggcgtctacaccgatgtggcctactacctggcctggatccgggagcacaccgtttcctgattgctcagggactcatctttccctccttggtgattccgcagtgagagagtggctggggcatggaaggcaagattgtgtcccattcccccagtgcggccagctccgcgccaggatggcgcaggaactcaataaagtgctttgaaaatgctgagaaaaaaaaaaa

SEQ ID NO: 2 - RNA, 19 nt, Artificial sequence
  F12 mRNA target sequence
caaggagcauaaguacaaa

SEQ ID NO: 3 - RNA, 19 nt, Artificial sequence
  F12 mRNA target sequence
uggagucaacacuuucgau

SEQ ID NO: 4 - RNA, 19 nt, Artificial sequence
  F12 mRNA target sequence
ggagucaacacuuucgauu

SEQ ID NO: 5 - RNA, 19 nt, Artificial sequence
  F12 mRNA target sequence
cccaaggagcauaaguaca

SEQ ID NO: 6 - RNA, 19 nt, Artificial sequence
  F12 mRNA target sequence
ccaaggagcauaaguacaa

SEQ ID NO: 7 - RNA, 19 nt, Artificial sequence
  F12 mRNA target sequence
aaggagcauaaguacaaag

SEQ ID NO: 8 - RNA, 19 nt, Artificial sequence
  F12 mRNA target sequence
agcauaaguacaaagcuga

SEQ ID NO: 9 - RNA, 19 nt, Artificial sequence
  F12 mRNA target sequence
ccacaaauguacccacaag

SEQ ID NO: 10 - RNA, 19 nt, Artificial sequence
  F12 mRNA target sequence
ccaagaaagugaaagacca

SEQ ID NO: 11 - RNA, 19 nt, Artificial sequence
  F12 mRNA target sequence
ggggucgcugccuagaggu

SEQ ID NO: 12 - RNA, 19 nt, Artificial sequence
  F12 mRNA target sequence
gccggaacccggacaacga

SEQ ID NO: 13 - RNA, 19 nt, Artificial sequence
  F12 mRNA target sequence
cggaacccggacaacgaca

SEQ ID NO: 14 - RNA, 19 nt, Artificial sequence
  F12 mRNA target sequence
ggaacccggacaacgacau

SEQ ID NO: 15 - RNA, 19 nt, Artificial sequence
  F12 mRNA target sequence
gcuccgcaagagucugucu

SEQ ID NO: 16 - RNA, 19 nt, Artificial sequence
  F12 mRNA target sequence
cgcaagagucugucuucga

SEQ ID NO: 17 - RNA, 19 nt, Artificial sequence
  F12 mRNA target sequence
cgcuccugucgccuuacgu

SEQ ID NO: 18 - RNA, 19 nt, Artificial sequence
  F12 mRNA target sequence
gcuccugucgccuuacguu

SEQ ID NO: 19 - RNA, 19 nt, Artificial sequence
  F12 mRNA target sequence
gcaacaagccaggcgucua

SEQ ID NO: 20 - RNA, 19 nt, Artificial sequence
  F12 mRNA target sequence
gaacucaauaaagugcuuu

SEQ ID NO: 21 - RNA, 19 nt, Artificial sequence
  F12 mRNA target sequence
cucaauaaagugcuuugaa

SEQ ID NO: 22 - RNA, 19 nt, Artificial sequence
  F12 mRNA target sequence
ucaauaaagugcuuugaaa

SEQ ID NO: 23 - RNA, 19 nt, Artificial sequence
  F12 RNAi agent antisense strand core stretch base sequence
uuuguacuuaugcuccuug

SEQ ID NO: 24 - RNA, 19 nt, Artificial sequence
  F12 RNAi agent antisense strand core stretch base sequence
  modified_base 1: n = any nucleotide
nuuguacuuaugcuccuug

SEQ ID NO: 25 - RNA, 19 nt, Artificial sequence
  F12 RNAi agent antisense strand core stretch base sequence
  modified_base 1, 19: n = any nucleotide
nuuguacuuaugcuccuun

SEQ ID NO: 26 - RNA, 19 nt, Artificial sequence
  F12 RNAi agent antisense strand core stretch base sequence
aucgaaaguguugacucca

SEQ ID NO: 27 - RNA, 19 nt, Artificial sequence
  F12 RNAi agent antisense strand core stretch base sequence
uucgaaaguguugacucca

SEQ ID NO: 28 - RNA, 19 nt, Artificial sequence
  F12 RNAi agent antisense strand core stretch base sequence
  modified_base 1: n = any nucleotide
nucgaaaguguugacucca

SEQ ID NO: 29 - RNA, 19 nt, Artificial sequence
  F12 RNAi agent antisense strand core stretch base sequence
  modified_base 1, 19: n = any nucleotide
nucgaaaguguugacuccn

SEQ ID NO: 30 - RNA, 19 nt, Artificial sequence
  F12 RNAi agent antisense strand core stretch base sequence
aaucgaaaguguugacucc

SEQ ID NO: 31 - RNA, 19 nt, Artificial sequence
  F12 RNAi agent antisense strand core stretch base sequence
uaucgaaaguguugacucc

SEQ ID NO: 32 - RNA, 19 nt, Artificial sequence
  F12 RNAi agent antisense strand core stretch base sequence
  modified_base 1: n = any nucleotide
naucgaaaguguugacucc

SEQ ID NO: 33 - RNA, 19 nt, Artificial sequence
  F12 RNAi agent antisense strand core stretch base sequence
  modified_base 1, 19: n = any nucleotide
naucgaaaguguugacucn

SEQ ID NO: 34 - RNA, 19 nt, Artificial sequence
  F12 RNAi agent antisense strand core stretch base sequence
uguacuuaugcuccuuggg

SEQ ID NO: 35 - RNA, 19 nt, Artificial sequence
  F12 RNAi agent antisense strand core stretch base sequence
  modified_base 1: n = any nucleotide
nguacuuaugcuccuuggg

SEQ ID NO: 36 - RNA, 19 nt, Artificial sequence
  F12 RNAi agent antisense strand core stretch base sequence
  modified_base 1, 19: n = any nucleotide
nguacuuaugcuccuuggn

SEQ ID NO: 37 - RNA, 19 nt, Artificial sequence
  F12 RNAi agent antisense strand core stretch base sequence
uuguacuuaugcuccuugg

SEQ ID NO: 38 - RNA, 19 nt, Artificial sequence
  F12 RNAi agent antisense strand core stretch base sequence
  modified_base 1: n = any nucleotide
nuguacuuaugcuccuugg

SEQ ID NO: 39 - RNA, 19 nt, Artificial sequence
  F12 RNAi agent antisense strand core stretch base sequence
  modified_base 1, 19: n = any nucleotide
nuguacuuaugcuccuugn

SEQ ID NO: 40 - RNA, 19 nt, Artificial sequence
  F12 RNAi agent antisense strand core stretch base sequence
cuuuguacuuaugcuccuu

SEQ ID NO: 41 - RNA, 19 nt, Artificial sequence
  F12 RNAi agent antisense strand core stretch base sequence
uuuuguacuuaugcuccuu

SEQ ID NO: 42 - RNA, 19 nt, Artificial sequence
  F12 RNAi agent antisense strand core stretch base sequence
  modified_base 1: n = any nucleotide
nuuuguacuuaugcuccuu

SEQ ID NO: 43 - RNA, 19 nt, Artificial sequence
  F12 RNAi agent antisense strand core stretch base sequence
  modified_base 1, 19: n = any nucleotide
nuuuguacuuaugcuccun

SEQ ID NO: 44 - RNA, 19 nt, Artificial sequence
  F12 RNAi agent antisense strand core stretch base sequence
ucagcuuuguacuuaugcu

SEQ ID NO: 45 - RNA, 19 nt, Artificial sequence
  F12 RNAi agent antisense strand core stretch base sequence
  modified_base 1: n = any nucleotide
ncagcuuuguacuuaugcu

SEQ ID NO: 46 - RNA, 19 nt, Artificial sequence
  F12 RNAi agent antisense strand core stretch base sequence
  modified_base 1, 19: n = any nucleotide
ncagcuuuguacuuaugcn

SEQ ID NO: 47 - RNA, 19 nt, Artificial sequence
  F12 RNAi agent antisense strand core stretch base sequence
cuuguggguacauuugugg

SEQ ID NO: 48 - RNA, 19 nt, Artificial sequence
  F12 RNAi agent antisense strand core stretch base sequence
uuuguggguacauuugugg

SEQ ID NO: 49 - RNA, 19 nt, Artificial sequence
  F12 RNAi agent antisense strand core stretch base sequence
  modified_base 1: n = any nucleotide
nuuguggguacauuugugg

SEQ ID NO: 50 - RNA, 19 nt, Artificial sequence
  F12 RNAi agent antisense strand core stretch base sequence
  modified_base 1, 19: n = any nucleotide
nuuguggguacauuugugn

SEQ ID NO: 51 - RNA, 19 nt, Artificial sequence
  F12 RNAi agent antisense strand core stretch base sequence
uggucuuucacuuucuugg

SEQ ID NO: 52 - RNA, 19 nt, Artificial sequence
  F12 RNAi agent antisense strand core stretch base sequence
  modified_base 1: n = any nucleotide
nggucuuucacuuucuugg

SEQ ID NO: 53 - RNA, 19 nt, Artificial sequence
  F12 RNAi agent antisense strand core stretch base sequence
  modified_base 1, 19: n = any nucleotide
nggucuuucacuuucuugn

SEQ ID NO: 54 - RNA, 19 nt, Artificial sequence
  F12 RNAi agent antisense strand core stretch base sequence
accucuaggcagcgacccc

SEQ ID NO: 55 - RNA, 19 nt, Artificial sequence
  F12 RNAi agent antisense strand core stretch base sequence
uccucuaggcagcgacccc

SEQ ID NO: 56 - RNA, 19 nt, Artificial sequence
  F12 RNAi agent antisense strand core stretch base sequence
  modified_base 1: n = any nucleotide
nccucuaggcagcgacccc

SEQ ID NO: 57 - RNA, 19 nt, Artificial sequence
  F12 RNAi agent antisense strand core stretch base sequence
  modified_base 1, 19: n = any nucleotide
nccucuaggcagcgacccn

SEQ ID NO: 58 - RNA, 19 nt, Artificial sequence
  F12 RNAi agent antisense strand core stretch base sequence
ucguuguccggguuccggc

SEQ ID NO: 59 - RNA, 19 nt, Artificial sequence
  F12 RNAi agent antisense strand core stretch base sequence
  modified_base 1: n = any nucleotide
ncguuguccggguuccggc

SEQ ID NO: 60 - RNA, 19 nt, Artificial sequence
  F12 RNAi agent antisense strand core stretch base sequence
  modified_base 1, 19: n = any nucleotide
ncguuguccggguuccggn

SEQ ID NO: 61 - RNA, 19 nt, Artificial sequence
  F12 RNAi agent antisense strand core stretch base sequence
ugucguuguccggguuccg

SEQ ID NO: 62 - RNA, 19 nt, Artificial sequence
  F12 RNAi agent antisense strand core stretch base sequence
  modified_base 1: n = any nucleotide
ngucguuguccggguuccg

SEQ ID NO: 63 - RNA, 19 nt, Artificial sequence
  F12 RNAi agent antisense strand core stretch base sequence
  modified_base 1, 19: n = any nucleotide
ngucguuguccggguuccn

SEQ ID NO: 64 - RNA, 19 nt, Artificial sequence
  F12 RNAi agent antisense strand core stretch base sequence
augucguuguccggguucc

SEQ ID NO: 65 - RNA, 19 nt, Artificial sequence
  F12 RNAi agent antisense strand core stretch base sequence
uugucguuguccggguucc

SEQ ID NO: 66 - RNA, 19 nt, Artificial sequence
  F12 RNAi agent antisense strand core stretch base sequence
  modified_base 1: n = any nucleotide
nugucguuguccggguucc

SEQ ID NO: 67 - RNA, 19 nt, Artificial sequence
  F12 RNAi agent antisense strand core stretch base sequence
  modified_base 1, 19: n = any nucleotide
nugucguuguccggguucn

SEQ ID NO: 68 - RNA, 19 nt, Artificial sequence
  F12 RNAi agent antisense strand core stretch base sequence
agacagacucuugcggagc

SEQ ID NO: 69 - RNA, 19 nt, Artificial sequence
  F12 RNAi agent antisense strand core stretch base sequence
ugacagacucuugcggagc

SEQ ID NO: 70 - RNA, 19 nt, Artificial sequence
  F12 RNAi agent antisense strand core stretch base sequence
  modified_base 1: n = any nucleotide
ngacagacucuugcggagc

SEQ ID NO: 71 - RNA, 19 nt, Artificial sequence
  F12 RNAi agent antisense strand core stretch base sequence
  modified_base 1, 19: n = any nucleotide
ngacagacucuugcggagn

SEQ ID NO: 72 - RNA, 19 nt, Artificial sequence
  F12 RNAi agent antisense strand core stretch base sequence
ucgaagacagacucuugcg

SEQ ID NO: 73 - RNA, 19 nt, Artificial sequence
  F12 RNAi agent antisense strand core stretch base sequence
  modified_base 1: n = any nucleotide
ncgaagacagacucuugcg

SEQ ID NO: 74 - RNA, 19 nt, Artificial sequence
  F12 RNAi agent antisense strand core stretch base sequence
  modified_base 1, 19: n = any nucleotide
ncgaagacagacucuugcn

SEQ ID NO: 75 - RNA, 19 nt, Artificial sequence
  F12 RNAi agent antisense strand core stretch base sequence
acguaaggcgacaggagcg

SEQ ID NO: 76 - RNA, 19 nt, Artificial sequence
  F12 RNAi agent antisense strand core stretch base sequence
ucguaaggcgacaggagcg

SEQ ID NO: 77 - RNA, 19 nt, Artificial sequence
  F12 RNAi agent antisense strand core stretch base sequence
  modified_base 1: n = any nucleotide
ncguaaggcgacaggagcg

SEQ ID NO: 78 - RNA, 19 nt, Artificial sequence
  F12 RNAi agent antisense strand core stretch base sequence
  modified_base 1, 19: n = any nucleotide
ncguaaggcgacaggagcn

SEQ ID NO: 79 - RNA, 19 nt, Artificial sequence
  F12 RNAi agent antisense strand core stretch base sequence
aacguaaggcgacaggagc

SEQ ID NO: 80 - RNA, 19 nt, Artificial sequence
  F12 RNAi agent antisense strand core stretch base sequence
uacguaaggcgacaggagc

SEQ ID NO: 81 - RNA, 19 nt, Artificial sequence
  F12 RNAi agent antisense strand core stretch base sequence
  modified_base 1: n = any nucleotide
nacguaaggcgacaggagc

SEQ ID NO: 82 - RNA, 19 nt, Artificial sequence
  F12 RNAi agent antisense strand core stretch base sequence
  modified_base 1, 19: n = any nucleotide
nacguaaggcgacaggagn

SEQ ID NO: 83 - RNA, 19 nt, Artificial sequence
  F12 RNAi agent antisense strand core stretch base sequence
uagacgccuggcuuguugc

SEQ ID NO: 84 - RNA, 19 nt, Artificial sequence
  F12 RNAi agent antisense strand core stretch base sequence
  modified_base 1: n = any nucleotide
nagacgccuggcuuguugc

SEQ ID NO: 85 - RNA, 19 nt, Artificial sequence
  F12 RNAi agent antisense strand core stretch base sequence
  modified_base 1, 19: n = any nucleotide
nagacgccuggcuuguugn

SEQ ID NO: 86 - RNA, 19 nt, Artificial sequence
  F12 RNAi agent antisense strand core stretch base sequence
aaagcacuuuauugaguuc

SEQ ID NO: 87 - RNA, 19 nt, Artificial sequence
  F12 RNAi agent antisense strand core stretch base sequence
uaagcacuuuauugaguuc

SEQ ID NO: 88 - RNA, 19 nt, Artificial sequence
  F12 RNAi agent antisense strand core stretch base sequence
  modified_base 1: n = any nucleotide
naagcacuuuauugaguuc

SEQ ID NO: 89 - RNA, 19 nt, Artificial sequence
  F12 RNAi agent antisense strand core stretch base sequence
  modified_base 1, 19: n = any nucleotide
naagcacuuuauugaguun

SEQ ID NO: 90 - RNA, 19 nt, Artificial sequence
  F12 RNAi agent antisense strand core stretch base sequence
uucaaagcacuuuauugag

SEQ ID NO: 91 - RNA, 19 nt, Artificial sequence
  F12 RNAi agent antisense strand core stretch base sequence
  modified_base 1: n = any nucleotide
nucaaagcacuuuauugag

SEQ ID NO: 92 - RNA, 19 nt, Artificial sequence
  F12 RNAi agent antisense strand core stretch base sequence
  modified_base 1, 19: n = any nucleotide
nucaaagcacuuuauugan

SEQ ID NO: 93 - RNA, 19 nt, Artificial sequence
  F12 RNAi agent antisense strand core stretch base sequence
uuucaaagcacuuuauuga

SEQ ID NO: 94 - RNA, 19 nt, Artificial sequence
  F12 RNAi agent antisense strand core stretch base sequence
  modified_base 1: n = any nucleotide
nuucaaagcacuuuauuga

SEQ ID NO: 95 - RNA, 19 nt, Artificial sequence
  F12 RNAi agent antisense strand core stretch base sequence
  modified_base 1, 19: n = any nucleotide
nuucaaagcacuuuauugn

SEQ ID NO: 96 - RNA, 19 nt, Artificial sequence
  F12 RNAi agent sense strand core stretch base sequence
caaggagcauaaguacaaa

SEQ ID NO: 97 - RNA, 19 nt, Artificial sequence
  F12 RNAi agent sense strand core stretch base sequence
  modified_base 19: n = any nucleotide
caaggagcauaaguacaan

SEQ ID NO: 98 - RNA, 19 nt, Artificial sequence
  F12 RNAi agent sense strand core stretch base sequence
  modified_base 1, 19: n = any nucleotide
naaggagcauaaguacaan

SEQ ID NO: 99 - RNA, 19 nt, Artificial sequence
  F12 RNAi agent sense strand core stretch base sequence
uggagucaacacuuucgau

SEQ ID NO: 100 - RNA, 19 nt, Artificial sequence
  F12 RNAi agent sense strand core stretch base sequence
uggagucaacacuuucgaa

SEQ ID NO: 101 - RNA, 19 nt, Artificial sequence
  F12 RNAi agent sense strand core stretch base sequence
  modified_base 19: n = any nucleotide
uggagucaacacuuucgan

SEQ ID NO: 102 - RNA, 19 nt, Artificial sequence
  F12 RNAi agent sense strand core stretch base sequence
  modified_base 1, 19: n = any nucleotide
nggagucaacacuuucgan

SEQ ID NO: 103 - RNA, 19 nt, Artificial sequence
  F12 RNAi agent sense strand core stretch base sequence
ggagucaacacuuucgauu

SEQ ID NO: 104 - RNA, 19 nt, Artificial sequence
  F12 RNAi agent sense strand core stretch base sequence
ggagucaacacuuucgaua

SEQ ID NO: 105 - RNA, 19 nt, Artificial sequence
  F12 RNAi agent sense strand core stretch base sequence
  modified_base 19: n = any nucleotide
ggagucaacacuuucgaun

SEQ ID NO: 106 - RNA, 19 nt, Artificial sequence
  F12 RNAi agent sense strand core stretch base sequence
  modified_base 1, 19: n = any nucleotide
ngagucaacacuuucgaun

SEQ ID NO: 107 - RNA, 19 nt, Artificial sequence
  F12 RNAi agent sense strand core stretch base sequence
cccaaggagcauaaguaca

SEQ ID NO: 108 - RNA, 19 nt, Artificial sequence
  F12 RNAi agent sense strand core stretch base sequence
  modified_base 19: n = any nucleotide
cccaaggagcauaaguacn

SEQ ID NO: 109 - RNA, 19 nt, Artificial sequence
  F12 RNAi agent sense strand core stretch base sequence
  modified_base 1, 19: n = any nucleotide
nccaaggagcauaaguacn

SEQ ID NO: 110 - RNA, 19 nt, Artificial sequence
  F12 RNAi agent sense strand core stretch base sequence
ccaaggagcauaaguacaa

SEQ ID NO: 111 - RNA, 19 nt, Artificial sequence
  F12 RNAi agent sense strand core stretch base sequence
  modified_base 19: n = any nucleotide
ccaaggagcauaaguacan

SEQ ID NO: 112 - RNA, 19 nt, Artificial sequence
  F12 RNAi agent sense strand core stretch base sequence
  modified_base 1, 19: n = any nucleotide
ncaaggagcauaaguacan

SEQ ID NO: 113 - RNA, 19 nt, Artificial sequence
  F12 RNAi agent sense strand core stretch base sequence
aaggagcauaaguacaaag

SEQ ID NO: 114 - RNA, 19 nt, Artificial sequence
  F12 RNAi agent sense strand core stretch base sequence
aaggagcauaaguacaaaa

SEQ ID NO: 115 - RNA, 19 nt, Artificial sequence
  F12 RNAi agent sense strand core stretch base sequence
  modified_base 19: n = any nucleotide
aaggagcauaaguacaaan

SEQ ID NO: 116 - RNA, 19 nt, Artificial sequence
  F12 RNAi agent sense strand core stretch base sequence
  modified_base 1, 19: n = any nucleotide
naggagcauaaguacaaan

SEQ ID NO: 117 - RNA, 19 nt, Artificial sequence
  F12 RNAi agent sense strand core stretch base sequence
agcauaaguacaaagcuga

SEQ ID NO: 118 - RNA, 19 nt, Artificial sequence
  F12 RNAi agent sense strand core stretch base sequence
  modified_base 19: n = any nucleotide
agcauaaguacaaagcugn

SEQ ID NO: 119 - RNA, 19 nt, Artificial sequence
  F12 RNAi agent sense strand core stretch base sequence
  modified_base 1, 19: n = any nucleotide
ngcauaaguacaaagcugn

SEQ ID NO: 120 - RNA, 19 nt, Artificial sequence
  F12 RNAi agent sense strand core stretch base sequence
ccacaaauguacccacaag

SEQ ID NO: 121 - RNA, 19 nt, Artificial sequence
  F12 RNAi agent sense strand core stretch base sequence
ccacaaauguacccacaaa

SEQ ID NO: 122 - RNA, 19 nt, Artificial sequence
  F12 RNAi agent sense strand core stretch base sequence
  modified_base 19: n = any nucleotide
ccacaaauguacccacaan

SEQ ID NO: 123 - RNA, 19 nt, Artificial sequence
  F12 RNAi agent sense strand core stretch base sequence
  modified_base 1, 19: n = any nucleotide
ncacaaauguacccacaan

SEQ ID NO: 124 - RNA, 19 nt, Artificial sequence
  F12 RNAi agent sense strand core stretch base sequence
ccaagaaagugaaagacca

SEQ ID NO: 125 - RNA, 19 nt, Artificial sequence
  F12 RNAi agent sense strand core stretch base sequence
  modified_base 19: n = any nucleotide
ccaagaaagugaaagaccn

SEQ ID NO: 126 - RNA, 19 nt, Artificial sequence
  F12 RNAi agent sense strand core stretch base sequence
  modified_base 1, 19: n = any nucleotide
ncaagaaagugaaagaccn

SEQ ID NO: 127 - RNA, 19 nt, Artificial sequence
  F12 RNAi agent sense strand core stretch base sequence
ggggucgcugccuagaggu

SEQ ID NO: 128 - RNA, 19 nt, Artificial sequence
  F12 RNAi agent sense strand core stretch base sequence
ggggucgcugccuagagga

SEQ ID NO: 129 - RNA, 19 nt, Artificial sequence
  F12 RNAi agent sense strand core stretch base sequence
  modified_base 19: n = any nucleotide
ggggucgcugccuagaggn

SEQ ID NO: 130 - RNA, 19 nt, Artificial sequence
  F12 RNAi agent sense strand core stretch base sequence
  modified_base 1, 19: n = any nucleotide
ngggucgcugccuagaggn

SEQ ID NO: 131 - RNA, 19 nt, Artificial sequence
  F12 RNAi agent sense strand core stretch base sequence
gccggaacccggacaacga

SEQ ID NO: 132 - RNA, 19 nt, Artificial sequence
  F12 RNAi agent sense strand core stretch base sequence
  modified_base 19: n = any nucleotide
gccggaacccggacaacgn

SEQ ID NO: 133 - RNA, 19 nt, Artificial sequence
  F12 RNAi agent sense strand core stretch base sequence
  modified_base 1, 19: n = any nucleotide
nccggaacccggacaacgn

SEQ ID NO: 134 - RNA, 19 nt, Artificial sequence
  F12 RNAi agent sense strand core stretch base sequence
cggaacccggacaacgaca

SEQ ID NO: 135 - RNA, 19 nt, Artificial sequence
  F12 RNAi agent sense strand core stretch base sequence
  modified_base 19: n = any nucleotide
cggaacccggacaacgacn

SEQ ID NO: 136 - RNA, 19 nt, Artificial sequence
  F12 RNAi agent sense strand core stretch base sequence
  modified_base 1, 19: n = any nucleotide
nggaacccggacaacgacn

SEQ ID NO: 137 - RNA, 19 nt, Artificial sequence
  F12 RNAi agent sense strand core stretch base sequence
ggaacccggacaacgacau

SEQ ID NO: 138 - RNA, 19 nt, Artificial sequence
  F12 RNAi agent sense strand core stretch base sequence
ggaacccggacaacgacaa

SEQ ID NO: 139 - RNA, 19 nt, Artificial sequence
  F12 RNAi agent sense strand core stretch base sequence
  modified_base 19: n = any nucleotide
ggaacccggacaacgacan

SEQ ID NO: 140 - RNA, 19 nt, Artificial sequence
  F12 RNAi agent sense strand core stretch base sequence
  modified_base 1, 19: n = any nucleotide
ngaacccggacaacgacan

SEQ ID NO: 141 - RNA, 19 nt, Artificial sequence
  F12 RNAi agent sense strand core stretch base sequence
gcuccgcaagagucugucu

SEQ ID NO: 142 - RNA, 19 nt, Artificial sequence
  F12 RNAi agent sense strand core stretch base sequence
gcuccgcaagagucuguca

SEQ ID NO: 143 - RNA, 19 nt, Artificial sequence
  F12 RNAi agent sense strand core stretch base sequence
  modified_base 19: n = any nucleotide
gcuccgcaagagucugucn

SEQ ID NO: 144 - RNA, 19 nt, Artificial sequence
  F12 RNAi agent sense strand core stretch base sequence
  modified_base 1, 19: n = any nucleotide
ncuccgcaagagucugucn

SEQ ID NO: 145 - RNA, 19 nt, Artificial sequence
  F12 RNAi agent sense strand core stretch base sequence
cgcaagagucugucuucga

SEQ ID NO: 146 - RNA, 19 nt, Artificial sequence
  F12 RNAi agent sense strand core stretch base sequence
  modified_base 19: n = any nucleotide
cgcaagagucugucuucgn

SEQ ID NO: 147 - RNA, 19 nt, Artificial sequence
  F12 RNAi agent sense strand core stretch base sequence
  modified_base 1, 19: n = any nucleotide
ngcaagagucugucuucgn

SEQ ID NO: 148 - RNA, 19 nt, Artificial sequence
  F12 RNAi agent sense strand core stretch base sequence
cgcuccugucgccuuacgu

SEQ ID NO: 149 - RNA, 19 nt, Artificial sequence
  F12 RNAi agent sense strand core stretch base sequence
cgcuccugucgccuuacga

SEQ ID NO: 150 - RNA, 19 nt, Artificial sequence
  F12 RNAi agent sense strand core stretch base sequence
  modified_base 19: n = any nucleotide
cgcuccugucgccuuacgn

SEQ ID NO: 151 - RNA, 19 nt, Artificial sequence
  F12 RNAi agent sense strand core stretch base sequence
  modified_base 1, 19: n = any nucleotide
ngcuccugucgccuuacgn

SEQ ID NO: 152 - RNA, 19 nt, Artificial sequence
  F12 RNAi agent sense strand core stretch base sequence
gcuccugucgccuuacguu

SEQ ID NO: 153 - RNA, 19 nt, Artificial sequence
  F12 RNAi agent sense strand core stretch base sequence
gcuccugucgccuuacgua

SEQ ID NO: 154 - RNA, 19 nt, Artificial sequence
  F12 RNAi agent sense strand core stretch base sequence
  modified_base 19: n = any nucleotide
gcuccugucgccuuacgun

SEQ ID NO: 155 - RNA, 19 nt, Artificial sequence
  F12 RNAi agent sense strand core stretch base sequence
  modified_base 1, 19: n = any nucleotide
ncuccugucgccuuacgun

SEQ ID NO: 156 - RNA, 19 nt, Artificial sequence
  F12 RNAi agent sense strand core stretch base sequence
gcaacaagccaggcgucua

SEQ ID NO: 157 - RNA, 19 nt, Artificial sequence
  F12 RNAi agent sense strand core stretch base sequence
  modified_base 19: n = any nucleotide
gcaacaagccaggcgucun

SEQ ID NO: 158 - RNA, 19 nt, Artificial sequence
  F12 RNAi agent sense strand core stretch base sequence
  modified_base 1, 19: n = any nucleotide
ncaacaagccaggcgucun

SEQ ID NO: 159 - RNA, 19 nt, Artificial sequence
  F12 RNAi agent sense strand core stretch base sequence
gaacucaauaaagugcuuu

SEQ ID NO: 160 - RNA, 19 nt, Artificial sequence
  F12 RNAi agent sense strand core stretch base sequence
gaacucaauaaagugcuua

SEQ ID NO: 161 - RNA, 19 nt, Artificial sequence
  F12 RNAi agent sense strand core stretch base sequence
  modified_base 19: n = any nucleotide
gaacucaauaaagugcuun

SEQ ID NO: 162 - RNA, 19 nt, Artificial sequence
  F12 RNAi agent sense strand core stretch base sequence
  modified_base 1, 19: n = any nucleotide
naacucaauaaagugcuun

SEQ ID NO: 163 - RNA, 19 nt, Artificial sequence
  F12 RNAi agent sense strand core stretch base sequence
cucaauaaagugcuuugaa

SEQ ID NO: 164 - RNA, 19 nt, Artificial sequence
  F12 RNAi agent sense strand core stretch base sequence
  modified_base 19: n = any nucleotide
cucaauaaagugcuuugan

SEQ ID NO: 165 - RNA, 19 nt, Artificial sequence
  F12 RNAi agent sense strand core stretch base sequence
  modified_base 1, 19: n = any nucleotide
nucaauaaagugcuuugan

SEQ ID NO: 166 - RNA, 19 nt, Artificial sequence
  F12 RNAi agent sense strand core stretch base sequence
ucaauaaagugcuuugaaa

SEQ ID NO: 167 - RNA, 19 nt, Artificial sequence
  F12 RNAi agent sense strand core stretch base sequence
  modified_base 19: n = any nucleotide
ucaauaaagugcuuugaan

SEQ ID NO: 168 - RNA, 19 nt, Artificial sequence
  F12 RNAi agent sense strand core stretch base sequence
  modified_base 1, 19: n = any nucleotide
ncaauaaagugcuuugaan

SEQ ID NO: 169 - RNA, 26 nt, Artificial sequence
  F12 RNAi agent antisense strand modified sequence
uggucuuucacuuucuugggcucuau

SEQ ID NO: 170 - RNA, 26 nt, Artificial sequence
  F12 RNAi agent antisense strand modified sequence
gcgaugcccaagaaagugaaagacca

SEQ ID NO: 171 - RNA, 23 nt, Artificial sequence
  F12 RNAi agent antisense strand modified sequence
uggucuuucacuuucuugggcuc

SEQ ID NO: 172 - RNA, 21 nt, Artificial sequence
  F12 RNAi agent antisense strand modified sequence
uggucuuucacuuucuugguu

SEQ ID NO: 173 - RNA, 26 nt, Artificial sequence
  F12 RNAi agent antisense strand modified sequence
uggucuuucacuuucuugggcauuca

SEQ ID NO: 174 - RNA, 26 nt, Artificial sequence
  F12 RNAi agent antisense strand modified sequence
uggucuuucacuuucuugggcaucgc

SEQ ID NO: 175 - RNA, 26 nt, Artificial sequence
  F12 RNAi agent antisense strand modified sequence
uggucuuucacuuucuugggcucuau

SEQ ID NO: 176 - RNA, 25 nt, Artificial sequence
  F12 RNAi agent antisense strand modified sequence
uggucuuucacuuucuugggcucgc

SEQ ID NO: 177 - RNA, 21 nt, Artificial sequence
  F12 RNAi agent antisense strand modified sequence
uggucuuucacuuucuugggc

SEQ ID NO: 178 - RNA, 25 nt, Artificial sequence
  F12 RNAi agent antisense strand modified sequence
uggucuuucacuuucuugggcucgc

SEQ ID NO: 179 - RNA, 25 nt, Artificial sequence
  F12 RNAi agent antisense strand modified sequence
uggucuuucacuuucuugggcuuau

SEQ ID NO: 180 - RNA, 25 nt, Artificial sequence
  F12 RNAi agent antisense strand modified sequence
ucaccuucuugggcuccaaacacgc

SEQ ID NO: 181 - RNA, 23 nt, Artificial sequence
  F12 RNAi agent antisense strand modified sequence
ucaccuucuugggcuccaaacac

SEQ ID NO: 182 - RNA, 21 nt, Artificial sequence
  F12 RNAi agent antisense strand modified sequence
ucaccuucuugggcuccaaac

SEQ ID NO: 183 - RNA, 23 nt, Artificial sequence
  F12 RNAi agent antisense strand modified sequence
uggucuuucacuuucuugggcuu

SEQ ID NO: 184 - RNA, 24 nt, Artificial sequence
  F12 RNAi agent antisense strand modified sequence
uggucuuucacuuucuugggcguu

SEQ ID NO: 185 - RNA, 21 nt, Artificial sequence
  F12 RNAi agent antisense strand modified sequence
uggucuuucacuuucuugguu

SEQ ID NO: 186 - RNA, 21 nt, Artificial sequence
  F12 RNAi agent antisense strand modified sequence
uggucuuucacuuucuugggu

SEQ ID NO: 187 - RNA, 21 nt, Artificial sequence
  F12 RNAi agent antisense strand modified sequence
uggucuuucacuuucuugguu

SEQ ID NO: 188 - RNA, 21 nt, Artificial sequence
  F12 RNAi agent antisense strand modified sequence
uggucuuucacuuucuugguu

SEQ ID NO: 189 - RNA, 26 nt, Artificial sequence
  F12 RNAi agent antisense strand modified sequence
uuggucuuucacuuucuugggcucgc

SEQ ID NO: 190 - RNA, 26 nt, Artificial sequence
  F12 RNAi agent antisense strand modified sequence
uuggucuuucacuuucuugggcucgc

SEQ ID NO: 191 - RNA, 26 nt, Artificial sequence
  F12 RNAi agent antisense strand modified sequence
uggucuuucacuuucuugggcaucgc

SEQ ID NO: 192 - RNA, 26 nt, Artificial sequence
  F12 RNAi agent antisense strand modified sequence
uggucuuucacuuucuugggcaucgc

SEQ ID NO: 193 - RNA, 26 nt, Artificial sequence
  F12 RNAi agent antisense strand modified sequence
uggucuuucacuuucuugggcaucgc

SEQ ID NO: 194 - RNA, 23 nt, Artificial sequence
  F12 RNAi agent antisense strand modified sequence
uggucuuucacuuucuugggcau

SEQ ID NO: 195 - RNA, 26 nt, Artificial sequence
  F12 RNAi agent antisense strand modified sequence
ucuuucacuuucuugggcuccaauca

SEQ ID NO: 196 - RNA, 21 nt, Artificial sequence
  F12 RNAi agent antisense strand modified sequence
ucuuucacuuucuugggcuuu

SEQ ID NO: 197 - RNA, 23 nt, Artificial sequence
  F12 RNAi agent antisense strand modified sequence
ucuuucacuuucuugggcuccuu

SEQ ID NO: 198 - RNA, 26 nt, Artificial sequence
  F12 RNAi agent antisense strand modified sequence
ugucuuucacuuucuugggcuccuca

SEQ ID NO: 199 - RNA, 21 nt, Artificial sequence
  F12 RNAi agent antisense strand modified sequence
ugucuuucacuuucuuggguu

SEQ ID NO: 200 - RNA, 23 nt, Artificial sequence
  F12 RNAi agent antisense strand modified sequence
ugucuuucacuuucuugggcuuu

SEQ ID NO: 201 - RNA, 26 nt, Artificial sequence
  F12 RNAi agent antisense strand modified sequence
uuggucuuucacuuucuugggcuuca

SEQ ID NO: 202 - RNA, 21 nt, Artificial sequence
  F12 RNAi agent antisense strand modified sequence
uuggucuuucacuuucuuguu

SEQ ID NO: 203 - RNA, 23 nt, Artificial sequence
  F12 RNAi agent antisense strand modified sequence
uuggucuuucacuuucuuggguu

SEQ ID NO: 204 - RNA, 26 nt, Artificial sequence
  F12 RNAi agent antisense strand modified sequence
ugaagcugaggcucaaagcacuuuca

SEQ ID NO: 205 - RNA, 21 nt, Artificial sequence
  F12 RNAi agent antisense strand modified sequence
ugaagcugaggcucaaagcuu

SEQ ID NO: 206 - RNA, 23 nt, Artificial sequence
  F12 RNAi agent antisense strand modified sequence
ugaagcugaggcucaaagcacuu

SEQ ID NO: 207 - RNA, 26 nt, Artificial sequence
  F12 RNAi agent antisense strand modified sequence
ugagaagcugaggcucaaagcacuca

SEQ ID NO: 208 - RNA, 21 nt, Artificial sequence
  F12 RNAi agent antisense strand modified sequence
ugagaagcugaggcucaaauu

SEQ ID NO: 209 - RNA, 23 nt, Artificial sequence
  F12 RNAi agent antisense strand modified sequence
ugagaagcugaggcucaaagcuu

SEQ ID NO: 210 - RNA, 26 nt, Artificial sequence
  F12 RNAi agent antisense strand modified sequence
uuuuucaaagcacuuuauugaguuca

SEQ ID NO: 211 - RNA, 21 nt, Artificial sequence
  F12 RNAi agent antisense strand modified sequence
uuuuucaaagcacuuuauuuu

SEQ ID NO: 212 - RNA, 23 nt, Artificial sequence
  F12 RNAi agent antisense strand modified sequence
uuuuucaaagcacuuuauugauu

SEQ ID NO: 213 - RNA, 26 nt, Artificial sequence
  F12 RNAi agent antisense strand modified sequence
uggucuuucacuuucuugggcucuca

SEQ ID NO: 214 - RNA, 21 nt, Artificial sequence
  F12 RNAi agent antisense strand modified sequence
uggucuuucacuuucuugguu

SEQ ID NO: 215 - RNA, 23 nt, Artificial sequence
  F12 RNAi agent antisense strand modified sequence
uggucuuucacuuucuugggcuu

SEQ ID NO: 216 - RNA, 26 nt, Artificial sequence
  F12 RNAi agent antisense strand modified sequence
uggucuuucacuuucuugggcucuca

SEQ ID NO: 217 - RNA, 26 nt, Artificial sequence
  F12 RNAi agent antisense strand modified sequence
uggucuuucacuuucuugggcucuca

SEQ ID NO: 218 - RNA, 26 nt, Artificial sequence
  F12 RNAi agent antisense strand modified sequence
uggucuuucacuuucuugggcacuau

SEQ ID NO: 219 - RNA, 26 nt, Artificial sequence
  F12 RNAi agent antisense strand modified sequence
uggucuuucacuuucuugggcacuca

SEQ ID NO: 220 - RNA, 26 nt, Artificial sequence
  F12 RNAi agent antisense strand modified sequence
uggucuuucacuuucuugggcaccgc

SEQ ID NO: 221 - RNA, 26 nt, Artificial sequence
  F12 RNAi agent antisense strand modified sequence
uggucuuucacuuucuugggcacuca

SEQ ID NO: 222 - RNA, 26 nt, Artificial sequence
  F12 RNAi agent antisense strand modified sequence
uggucuuucacuuucuugggcaccgc

SEQ ID NO: 223 - RNA, 26 nt, Artificial sequence
  F12 RNAi agent antisense strand modified sequence
uggucuuucacuuucuugggcacuau

SEQ ID NO: 224 - RNA, 26 nt, Artificial sequence
  F12 RNAi agent antisense strand modified sequence
uggucuuucacuuucuugggcaccaa

SEQ ID NO: 225 - RNA, 26 nt, Artificial sequence
  F12 RNAi agent antisense strand modified sequence
uggucuuucacuuucuugggcaccuu

SEQ ID NO: 226 - RNA, 26 nt, Artificial sequence
  F12 RNAi agent antisense strand modified sequence
uggucuuucacuuucuugggcaccac

SEQ ID NO: 227 - RNA, 26 nt, Artificial sequence
  F12 RNAi agent antisense strand modified sequence
uggucuuucacuuucuugggcaccuc

SEQ ID NO: 228 - RNA, 23 nt, Artificial sequence
  F12 RNAi agent antisense strand modified sequence
uggucuuucacuuucuugggcuu

SEQ ID NO: 229 - RNA, 21 nt, Artificial sequence
  F12 RNAi agent antisense strand modified sequence
uggucuuucacuuucuugggc

SEQ ID NO: 230 - RNA, 24 nt, Artificial sequence
  F12 RNAi agent antisense strand modified sequence
uggucuuucacuuucuugggcauc

SEQ ID NO: 231 - RNA, 24 nt, Artificial sequence
  F12 RNAi agent antisense strand modified sequence
uggucuuucacuuucuugggcauc

SEQ ID NO: 232 - RNA, 23 nt, Artificial sequence
  F12 RNAi agent antisense strand modified sequence
uggucuuucacuuucuuggguuu

SEQ ID NO: 233 - RNA, 21 nt, Artificial sequence
  F12 RNAi agent antisense strand modified sequence
uggucuuucacuuucuuggga

SEQ ID NO: 234 - RNA, 21 nt, Artificial sequence
  F12 RNAi agent antisense strand modified sequence
uggucuuucacuuucaugggu

SEQ ID NO: 235 - RNA, 21 nt, Artificial sequence
  F12 RNAi agent antisense strand modified sequence
uggucuuucacuuucaugggu

SEQ ID NO: 236 - RNA, 21 nt, Artificial sequence
  F12 RNAi agent antisense strand modified sequence
aggucuuucacuuucaugggu

SEQ ID NO: 237 - RNA, 23 nt, Artificial sequence
  F12 RNAi agent antisense strand modified sequence
uggucuuucacuuucauggguuu

SEQ ID NO: 238 - RNA, 21 nt, Artificial sequence
  F12 RNAi agent antisense strand modified sequence
uggucuuucacuuucuugggu

SEQ ID NO: 239 - RNA, 24 nt, Artificial sequence
  F12 RNAi agent antisense strand modified sequence
ucuuucacuuucuugggcuccaaa

SEQ ID NO: 240 - RNA, 23 nt, Artificial sequence
  F12 RNAi agent antisense strand modified sequence
ucuuucacuuucuugggcuccaa

SEQ ID NO: 241 - RNA, 22 nt, Artificial sequence
  F12 RNAi agent antisense strand modified sequence
ucuuucacuuucuugggcucca

SEQ ID NO: 242 - RNA, 21 nt, Artificial sequence
  F12 RNAi agent antisense strand modified sequence
ucuuucacuuucuugggcucc

SEQ ID NO: 243 - RNA, 20 nt, Artificial sequence
  F12 RNAi agent antisense strand modified sequence
ucuuucacuuucuugggcuc

SEQ ID NO: 244 - RNA, 19 nt, Artificial sequence
  F12 RNAi agent antisense strand modified sequence
ucuuucacuuucuugggcu

SEQ ID NO: 245 - RNA, 24 nt, Artificial sequence
  F12 RNAi agent antisense strand modified sequence
ugucuuucacuuucuugggcucca

SEQ ID NO: 246 - RNA, 23 nt, Artificial sequence
  F12 RNAi agent antisense strand modified sequence
ugucuuucacuuucuugggcucc

SEQ ID NO: 247 - RNA, 22 nt, Artificial sequence
  F12 RNAi agent antisense strand modified sequence
ugucuuucacuuucuugggcuc

SEQ ID NO: 248 - RNA, 21 nt, Artificial sequence
  F12 RNAi agent antisense strand modified sequence
ugucuuucacuuucuugggcu

SEQ ID NO: 249 - RNA, 20 nt, Artificial sequence
  F12 RNAi agent antisense strand modified sequence
ugucuuucacuuucuugggc

SEQ ID NO: 250 - RNA, 19 nt, Artificial sequence
  F12 RNAi agent antisense strand modified sequence
ugucuuucacuuucuuggg

SEQ ID NO: 251 - RNA, 26 nt, Artificial sequence
  F12 RNAi agent antisense strand modified sequence
uggucuuucacuuucuugggcuccaa

SEQ ID NO: 252 - RNA, 24 nt, Artificial sequence
  F12 RNAi agent antisense strand modified sequence
uggucuuucacuuucuugggcucc

SEQ ID NO: 253 - RNA, 23 nt, Artificial sequence
  F12 RNAi agent antisense strand modified sequence
uggucuuucacuuucuugggcuc

SEQ ID NO: 254 - RNA, 22 nt, Artificial sequence
  F12 RNAi agent antisense strand modified sequence
uggucuuucacuuucuugggcu

SEQ ID NO: 255 - RNA, 21 nt, Artificial sequence
  F12 RNAi agent antisense strand modified sequence
uggucuuucacuuucuugggc

SEQ ID NO: 256 - RNA, 20 nt, Artificial sequence
  F12 RNAi agent antisense strand modified sequence
uggucuuucacuuucuuggg

SEQ ID NO: 257 - RNA, 19 nt, Artificial sequence
  F12 RNAi agent antisense strand modified sequence
uggucuuucacuuucuugg

SEQ ID NO: 258 - RNA, 24 nt, Artificial sequence
  F12 RNAi agent antisense strand modified sequence
uuggucuuucacuuucuugggcuc

SEQ ID NO: 259 - RNA, 23 nt, Artificial sequence
  F12 RNAi agent antisense strand modified sequence
uuggucuuucacuuucuugggcu

SEQ ID NO: 260 - RNA, 22 nt, Artificial sequence
  F12 RNAi agent antisense strand modified sequence
uuggucuuucacuuucuugggc

SEQ ID NO: 261 - RNA, 21 nt, Artificial sequence
  F12 RNAi agent antisense strand modified sequence
uuggucuuucacuuucuuggg

SEQ ID NO: 262 - RNA, 20 nt, Artificial sequence
  F12 RNAi agent antisense strand modified sequence
uuggucuuucacuuucuugg

SEQ ID NO: 263 - RNA, 19 nt, Artificial sequence
  F12 RNAi agent antisense strand modified sequence
uuggucuuucacuuucuug

SEQ ID NO: 264 - RNA, 24 nt, Artificial sequence
  F12 RNAi agent antisense strand modified sequence
ugaagcugaggcucaaagcacuuc

SEQ ID NO: 265 - RNA, 23 nt, Artificial sequence
  F12 RNAi agent antisense strand modified sequence
ugaagcugaggcucaaagcacuu

SEQ ID NO: 266 - RNA, 22 nt, Artificial sequence
  F12 RNAi agent antisense strand modified sequence
ugaagcugaggcucaaagcacu

SEQ ID NO: 267 - RNA, 21 nt, Artificial sequence
  F12 RNAi agent antisense strand modified sequence
ugaagcugaggcucaaagcac

SEQ ID NO: 268 - RNA, 20 nt, Artificial sequence
  F12 RNAi agent antisense strand modified sequence
ugaagcugaggcucaaagca

SEQ ID NO: 269 - RNA, 19 nt, Artificial sequence
  F12 RNAi agent antisense strand modified sequence
ugaagcugaggcucaaagc

SEQ ID NO: 270 - RNA, 24 nt, Artificial sequence
  F12 RNAi agent antisense strand modified sequence
ugagaagcugaggcucaaagcacu

SEQ ID NO: 271 - RNA, 23 nt, Artificial sequence
  F12 RNAi agent antisense strand modified sequence
ugagaagcugaggcucaaagcac

SEQ ID NO: 272 - RNA, 22 nt, Artificial sequence
  F12 RNAi agent antisense strand modified sequence
ugagaagcugaggcucaaagca

SEQ ID NO: 273 - RNA, 21 nt, Artificial sequence
  F12 RNAi agent antisense strand modified sequence
ugagaagcugaggcucaaagc

SEQ ID NO: 274 - RNA, 20 nt, Artificial sequence
  F12 RNAi agent antisense strand modified sequence
ugagaagcugaggcucaaag

SEQ ID NO: 275 - RNA, 19 nt, Artificial sequence
  F12 RNAi agent antisense strand modified sequence
ugagaagcugaggcucaaa

SEQ ID NO: 276 - RNA, 24 nt, Artificial sequence
  F12 RNAi agent antisense strand modified sequence
uuuuucaaagcacuuuauugaguu

SEQ ID NO: 277 - RNA, 23 nt, Artificial sequence
  F12 RNAi agent antisense strand modified sequence
uuuuucaaagcacuuuauugagu

SEQ ID NO: 278 - RNA, 22 nt, Artificial sequence
  F12 RNAi agent antisense strand modified sequence
uuuuucaaagcacuuuauugag

SEQ ID NO: 279 - RNA, 21 nt, Artificial sequence
  F12 RNAi agent antisense strand modified sequence
uuuuucaaagcacuuuauuga

SEQ ID NO: 280 - RNA, 20 nt, Artificial sequence
  F12 RNAi agent antisense strand modified sequence
uuuuucaaagcacuuuauug

SEQ ID NO: 281 - RNA, 19 nt, Artificial sequence
  F12 RNAi agent antisense strand modified sequence
uuuuucaaagcacuuuauu

SEQ ID NO: 282 - RNA, 24 nt, Artificial sequence
  F12 RNAi agent antisense strand modified sequence
uggucuuucacuuucuugggcauc

SEQ ID NO: 283 - RNA, 21 nt, Artificial sequence
  F12 RNAi agent antisense strand modified sequence
uggucuuucacuuucaugggu

SEQ ID NO: 284 - RNA, 23 nt, Artificial sequence
  F12 RNAi agent antisense strand modified sequence
uggucuuucacuuucuugggcuc

SEQ ID NO: 285 - RNA, 23 nt, Artificial sequence
  F12 RNAi agent antisense strand modified sequence
uggucuuucacuuucuugggcuc

SEQ ID NO: 286 - RNA, 21 nt, Artificial sequence
  F12 RNAi agent antisense strand modified sequence
uggucuuucacuuucuugggc

SEQ ID NO: 287 - RNA, 26 nt, Artificial sequence
  F12 RNAi agent antisense strand modified sequence
uggucuuucacuuucuugggcuccgc

SEQ ID NO: 288 - RNA, 23 nt, Artificial sequence
  F12 RNAi agent antisense strand modified sequence
uggucuuucacuuucuugggcuu

SEQ ID NO: 289 - RNA, 21 nt, Artificial sequence
  F12 RNAi agent antisense strand modified sequence
uggucuuucacuuucuugguu

SEQ ID NO: 290 - RNA, 21 nt, Artificial sequence
  F12 RNAi agent antisense strand modified sequence
uggucuuucacuuucuugggc

SEQ ID NO: 291 - RNA, 26 nt, Artificial sequence
  F12 RNAi agent antisense strand modified sequence
uuuuucaaagcacuuuauugaguuca

SEQ ID NO: 292 - RNA, 26 nt, Artificial sequence
  F12 RNAi agent antisense strand modified sequence
uuuuucaaagcacuuuauugaguuca

SEQ ID NO: 293 - RNA, 26 nt, Artificial sequence
  F12 RNAi agent antisense strand modified sequence
auuuucaaagcacuuuauugaguuca

SEQ ID NO: 294 - RNA, 23 nt, Artificial sequence
  F12 RNAi agent antisense strand modified sequence
uuuuucaaagcacuuuauugagu

SEQ ID NO: 295 - RNA, 21 nt, Artificial sequence
  F12 RNAi agent antisense strand modified sequence
uuuuucaaagcacuuuauuga

SEQ ID NO: 296 - RNA, 21 nt, Artificial sequence
  F12 RNAi agent antisense strand modified sequence
uuuuucaaagcacuuuauugc

SEQ ID NO: 297 - RNA, 21 nt, Artificial sequence
  F12 RNAi agent antisense strand modified sequence
uuuuucaaagcacuuuaucga

SEQ ID NO: 298 - RNA, 21 nt, Artificial sequence
  F12 RNAi agent antisense strand modified sequence
ugaagcugaggcucaaagcuu

SEQ ID NO: 299 - RNA, 21 nt, Artificial sequence
  F12 RNAi agent antisense strand modified sequence
ugaagcugaggcucaaagcac

SEQ ID NO: 300 - RNA, 21 nt, Artificial sequence
  F12 RNAi agent antisense strand modified sequence
uaagcacuuuauugaguuccu

SEQ ID NO: 301 - RNA, 22 nt, Artificial sequence
  F12 RNAi agent antisense strand modified sequence
uaagcacuuuauugaguuccuu

SEQ ID NO: 302 - RNA, 21 nt, Artificial sequence
  F12 RNAi agent antisense strand modified sequence
ucaaagcacuuuauugaguuc

SEQ ID NO: 303 - RNA, 22 nt, Artificial sequence
  F12 RNAi agent antisense strand modified sequence
ucaaagcacuuuauugaguucu

SEQ ID NO: 304 - RNA, 21 nt, Artificial sequence
  F12 RNAi agent antisense strand modified sequence
uucaaagcacuuuauugaguu

SEQ ID NO: 305 - RNA, 22 nt, Artificial sequence
  F12 RNAi agent antisense strand modified sequence
uucaaagcacuuuauugaguuc

SEQ ID NO: 306 - RNA, 23 nt, Artificial sequence
  F12 RNAi agent antisense strand modified sequence
uucaaagcacuuuauugaguucu

SEQ ID NO: 307 - RNA, 21 nt, Artificial sequence
  F12 RNAi agent antisense strand modified sequence
uuucaaagcacuauauugagu

SEQ ID NO: 308 - RNA, 21 nt, Artificial sequence
  F12 RNAi agent antisense strand modified sequence
auucaaagcacuauauugagu

SEQ ID NO: 309 - RNA, 23 nt, Artificial sequence
  F12 RNAi agent antisense strand modified sequence
uuucaaagcacuauauugaguuc

SEQ ID NO: 310 - RNA, 26 nt, Artificial sequence
  F12 RNAi agent antisense strand modified sequence
uuuuucaaagcacuuuauugaguuau

SEQ ID NO: 311 - RNA, 21 nt, Artificial sequence
  F12 RNAi agent antisense strand modified sequence
uggucuuucacuuucuugggc

SEQ ID NO: 312 - RNA, 22 nt, Artificial sequence
  F12 RNAi agent antisense strand modified sequence
uggucuuucacuuucuugggca

SEQ ID NO: 313 - RNA, 21 nt, Artificial sequence
  F12 RNAi agent antisense strand modified sequence
uaagcacuuuauugaguuccu

SEQ ID NO: 314 - RNA, 21 nt, Artificial sequence
  F12 RNAi agent antisense strand modified sequence
ucaaagcacuuuauugaguuc

SEQ ID NO: 315 - RNA, 21 nt, Artificial sequence
  F12 RNAi agent antisense strand modified sequence
uucaaagcacuuuauugaguu

SEQ ID NO: 316 - RNA, 21 nt, Artificial sequence
  F12 RNAi agent antisense strand modified sequence
uuucaaagcacuauauugagu

SEQ ID NO: 317 - RNA, 21 nt, Artificial sequence
  F12 RNAi agent antisense strand modified sequence
uuuuucaaagcacuuuauugu

SEQ ID NO: 318 - RNA, 21 nt, Artificial sequence
  F12 RNAi agent antisense strand modified sequence
uuuuucaaagcacuuuauugu

SEQ ID NO: 319 - RNA, 21 nt, Artificial sequence
  F12 RNAi agent antisense strand modified sequence
uuucaaagcacuuuauugagu

SEQ ID NO: 320 - RNA, 21 nt, Artificial sequence
  F12 RNAi agent antisense strand modified sequence
auucaaagcacuuuauugagu

SEQ ID NO: 321 - RNA, 23 nt, Artificial sequence
  F12 RNAi agent antisense strand modified sequence
uuucaaagcacuuuauugaguuc

SEQ ID NO: 322 - RNA, 21 nt, Artificial sequence
  F12 RNAi agent antisense strand modified sequence
uuucaaagcacuuuauugagu

SEQ ID NO: 323 - RNA, 22 nt, Artificial sequence
  F12 RNAi agent antisense strand modified sequence
uggucuuucacuuucuugggcu

SEQ ID NO: 324 - RNA, 23 nt, Artificial sequence
  F12 RNAi agent antisense strand modified sequence
uggucuuucacuuucuugggcuu

SEQ ID NO: 325 - RNA, 21 nt, Artificial sequence
  F12 RNAi agent antisense strand modified sequence
uggucuuucacuuucuugguc

SEQ ID NO: 326 - RNA, 21 nt, Artificial sequence
  F12 RNAi agent antisense strand modified sequence
uggucuuucacuuucuugguu

SEQ ID NO: 327 - RNA, 21 nt, Artificial sequence
  F12 RNAi agent antisense strand modified sequence
uuucaaagcacuuuauugagu

SEQ ID NO: 328 - RNA, 21 nt, Artificial sequence
  F12 RNAi agent antisense strand modified sequence
uuucaaagcacuuuauugagc

SEQ ID NO: 329 - RNA, 21 nt, Artificial sequence
  F12 RNAi agent antisense strand modified sequence
uucaaagcacuuuauugaguc

SEQ ID NO: 330 - RNA, 21 nt, Artificial sequence
  F12 RNAi agent antisense strand modified sequence
uucaaagcacuuuauugagcu

SEQ ID NO: 331 - RNA, 21 nt, Artificial sequence
  F12 RNAi agent antisense strand modified sequence
uucaaagcacuuuauugagcc

SEQ ID NO: 332 - RNA, 21 nt, Artificial sequence
  F12 RNAi agent antisense strand modified sequence
uucaaagcacuuuauugaguu

SEQ ID NO: 333 - RNA, 21 nt, Artificial sequence
  F12 RNAi agent antisense strand modified sequence
uucaaagcacuuuauugaguu

SEQ ID NO: 334 - RNA, 22 nt, Artificial sequence
  F12 RNAi agent antisense strand modified sequence
uucaaagcacuuuauugagucc

SEQ ID NO: 335 - RNA, 21 nt, Artificial sequence
  F12 RNAi agent antisense strand modified sequence
uucaaagcacuuuauugaguu

SEQ ID NO: 336 - RNA, 21 nt, Artificial sequence
  F12 RNAi agent antisense strand modified sequence
uucaaagcacuuuauugagcc

SEQ ID NO: 337 - RNA, 21 nt, Artificial sequence
  F12 RNAi agent antisense strand modified sequence
uucaaagcacuuuauugaguu

SEQ ID NO: 338 - RNA, 21 nt, Artificial sequence
  F12 RNAi agent antisense strand modified sequence
uuucaaagcacuuuauugagu

SEQ ID NO: 339 - RNA, 22 nt, Artificial sequence
  F12 RNAi agent antisense strand modified sequence
uuucaaagcacuuuauugaguu

SEQ ID NO: 340 - RNA, 22 nt, Artificial sequence
  F12 RNAi agent antisense strand modified sequence
uuucaaagcacuuuauugagcu

SEQ ID NO: 341 - RNA, 22 nt, Artificial sequence
  F12 RNAi agent antisense strand modified sequence
uuucaaagcacuuuauugaguc

SEQ ID NO: 342 - RNA, 23 nt, Artificial sequence
  F12 RNAi agent antisense strand modified sequence
uuucaaagcacuuuauugagucc

SEQ ID NO: 343 - RNA, 23 nt, Artificial sequence
  F12 RNAi agent antisense strand modified sequence
uuucaaagcacuuuauugaguuc

SEQ ID NO: 344 - RNA, 21 nt, Artificial sequence
  F12 RNAi agent antisense strand modified sequence
uuucaaagcacuuuauugagu

SEQ ID NO: 345 - RNA, 21 nt, Artificial sequence
  F12 RNAi agent antisense strand modified sequence
uuucaaagcacuuuauugauu

SEQ ID NO: 346 - RNA, 22 nt, Artificial sequence
  F12 RNAi agent antisense strand modified sequence
uuucaaagcacuuuauugagcc

SEQ ID NO: 347 - RNA, 21 nt, Artificial sequence
  F12 RNAi agent antisense strand modified sequence
uuucaaagcacuuuauugagu

SEQ ID NO: 348 - RNA, 21 nt, Artificial sequence
  F12 RNAi agent antisense strand modified sequence
uuucaaagcacuuuauugauu

SEQ ID NO: 349 - RNA, 21 nt, Artificial sequence
  F12 RNAi agent antisense strand modified sequence
uuucaaagcacuuuauugagu

SEQ ID NO: 350 - RNA, 23 nt, Artificial sequence
  F12 RNAi agent antisense strand modified sequence
uuucaaagcacuuuauugaguuc

SEQ ID NO: 351 - RNA, 21 nt, Artificial sequence
  F12 RNAi agent antisense strand modified sequence
uaagcacuuuauugaguuccc

SEQ ID NO: 352 - RNA, 21 nt, Artificial sequence
  F12 RNAi agent antisense strand modified sequence
aaagcacuuuauugaguuccu

SEQ ID NO: 353 - RNA, 21 nt, Artificial sequence
  F12 RNAi agent antisense strand modified sequence
uaagcacuuuauugaguuccu

SEQ ID NO: 354 - RNA, 22 nt, Artificial sequence
  F12 RNAi agent antisense strand modified sequence
uaagcacuuuauugaguuccug

SEQ ID NO: 355 - RNA, 21 nt, Artificial sequence
  F12 RNAi agent antisense strand modified sequence
uaagcacuuuauugaguuccu

SEQ ID NO: 356 - RNA, 21 nt, Artificial sequence
  F12 RNAi agent antisense strand modified sequence
uaagcacuuuauugaguuccu

SEQ ID NO: 357 - RNA, 21 nt, Artificial sequence
  F12 RNAi agent antisense strand modified sequence
uaagcacuuuauugaguuccu

SEQ ID NO: 358 - RNA, 21 nt, Artificial sequence
  F12 RNAi agent antisense strand modified sequence
uucaaagcacuuuauugaguu

SEQ ID NO: 359 - RNA, 22 nt, Artificial sequence
  F12 RNAi agent antisense strand modified sequence
uucaaagcacuuuauugaguuc

SEQ ID NO: 360 - RNA, 23 nt, Artificial sequence
  F12 RNAi agent antisense strand modified sequence
uggucuuucacuuucuugggcuc

SEQ ID NO: 361 - RNA, 23 nt, Artificial sequence
  F12 RNAi agent antisense strand modified sequence
uggucuuucacuuucuugggcuc

SEQ ID NO: 362 - RNA, 23 nt, Artificial sequence
  F12 RNAi agent antisense strand modified sequence
uggucuuucacuuucuugggcuc

SEQ ID NO: 363 - RNA, 23 nt, Artificial sequence
  F12 RNAi agent antisense strand modified sequence
uucaaagcacuuuauugaguucc

SEQ ID NO: 364 - RNA, 23 nt, Artificial sequence
  F12 RNAi agent antisense strand modified sequence
uucaaagcacuuuauugaguucc

SEQ ID NO: 365 - RNA, 23 nt, Artificial sequence
  F12 RNAi agent antisense strand modified sequence
uucaaagcacuuuauugaguucc

SEQ ID NO: 366 - RNA, 23 nt, Artificial sequence
  F12 RNAi agent antisense strand modified sequence
uucaaagcacuuuauugaguucc

SEQ ID NO: 367 - RNA, 23 nt, Artificial sequence
  F12 RNAi agent antisense strand modified sequence
uuucacuuucuugggcuccaaac

SEQ ID NO: 368 - RNA, 23 nt, Artificial sequence
  F12 RNAi agent antisense strand modified sequence
uuucacuuucuugggcuccaaac

SEQ ID NO: 369 - RNA, 23 nt, Artificial sequence
  F12 RNAi agent antisense strand modified sequence
uuucacuuucuugggcuccaaac

SEQ ID NO: 370 - RNA, 23 nt, Artificial sequence
  F12 RNAi agent antisense strand modified sequence
uuucacuuucuugggcuccaaac

SEQ ID NO: 371 - RNA, 21 nt, Artificial sequence
  F12 RNAi agent antisense strand modified sequence
uuucacuuucuugggcuccaa

SEQ ID NO: 372 - RNA, 21 nt, Artificial sequence
  F12 RNAi agent antisense strand modified sequence
uuucacuuucuugggcuccaa

SEQ ID NO: 373 - RNA, 21 nt, Artificial sequence
  F12 RNAi agent antisense strand modified sequence
uuucacuuucuugggcuccuu

SEQ ID NO: 374 - RNA, 21 nt, Artificial sequence
  F12 RNAi agent antisense strand modified sequence
uucaaagcacuuuauugaguu

SEQ ID NO: 375 - RNA, 21 nt, Artificial sequence
  F12 RNAi agent antisense strand modified sequence
uuuguacuuaugcuccuuggg

SEQ ID NO: 376 - RNA, 21 nt, Artificial sequence
  F12 RNAi agent antisense strand modified sequence
uaucgaaaguguugacuccaa

SEQ ID NO: 377 - RNA, 21 nt, Artificial sequence
  F12 RNAi agent antisense strand modified sequence
uuguacuuaugcuccuugguu

SEQ ID NO: 378 - RNA, 21 nt, Artificial sequence
  F12 RNAi agent antisense strand modified sequence
ucgaagacagacucuugcguu

SEQ ID NO: 379 - RNA, 21 nt, Artificial sequence
  F12 RNAi agent antisense strand modified sequence
uucaaagcacuuuauugaguu

SEQ ID NO: 380 - RNA, 23 nt, Artificial sequence
  F12 RNAi agent antisense strand modified sequence
uucaaagcacuuuauugaguucu

SEQ ID NO: 381 - RNA, 24 nt, Artificial sequence
  F12 RNAi agent antisense strand modified sequence
uucaaagcacuuuauugaguucuu

SEQ ID NO: 382 - RNA, 21 nt, Artificial sequence
  F12 RNAi agent antisense strand modified sequence
uucaaagcacuuuauugaguu

SEQ ID NO: 383 - RNA, 21 nt, Artificial sequence
  F12 RNAi agent antisense strand modified sequence
uaucgaaaguguugacuccuu

SEQ ID NO: 384 - RNA, 21 nt, Artificial sequence
  F12 RNAi agent antisense strand modified sequence
uaucgaaaguguugacuccuu

SEQ ID NO: 385 - RNA, 22 nt, Artificial sequence
  F12 RNAi agent antisense strand modified sequence
uaucgaaaguguugacuccaag

SEQ ID NO: 386 - RNA, 21 nt, Artificial sequence
  F12 RNAi agent antisense strand modified sequence
uuguacuuaugcuccuugggg

SEQ ID NO: 387 - RNA, 23 nt, Artificial sequence
  F12 RNAi agent antisense strand modified sequence
uuuguacuuaugcuccuuggguu

SEQ ID NO: 388 - RNA, 21 nt, Artificial sequence
  F12 RNAi agent antisense strand modified sequence
uuuguacuuaugcuccuuggg

SEQ ID NO: 389 - RNA, 21 nt, Artificial sequence
  F12 RNAi agent antisense strand modified sequence
uuuguacuuaugcuccuuguu

SEQ ID NO: 390 - RNA, 21 nt, Artificial sequence
  F12 RNAi agent antisense strand modified sequence
uuuguacuuaugcuccuuggg

SEQ ID NO: 391 - RNA, 22 nt, Artificial sequence
  F12 RNAi agent antisense strand modified sequence
uuuguacuuaugcuccuugggg

SEQ ID NO: 392 - RNA, 23 nt, Artificial sequence
  F12 RNAi agent antisense strand modified sequence
uuuguacuuaugcuccuuggggu

SEQ ID NO: 393 - RNA, 21 nt, Artificial sequence
  F12 RNAi agent antisense strand modified sequence
uuguacuuaugcuccuugggg

SEQ ID NO: 394 - RNA, 22 nt, Artificial sequence
  F12 RNAi agent antisense strand modified sequence
uuguacuuaugcuccuuggguu

SEQ ID NO: 395 - RNA, 23 nt, Artificial sequence
  F12 RNAi agent antisense strand modified sequence
uaucgaaaguguugacuccaagc

SEQ ID NO: 396 - RNA, 21 nt, Artificial sequence
  F12 RNAi agent antisense strand modified sequence
uuuguacuuaugcuccuuggg

SEQ ID NO: 397 - RNA, 21 nt, Artificial sequence
  F12 RNAi agent antisense strand modified sequence
uuuguacuuaugcuccuuggg

SEQ ID NO: 398 - RNA, 21 nt, Artificial sequence
  F12 RNAi agent antisense strand modified sequence
uuuguacuuaugcuccuuggu

SEQ ID NO: 399 - RNA, 20 nt, Artificial sequence
  F12 RNAi agent antisense strand modified sequence
uuuguacuuaugcuccuugg

SEQ ID NO: 400 - RNA, 21 nt, Artificial sequence
  F12 RNAi agent antisense strand modified sequence
uuuguacuuaugcuccuuguu

SEQ ID NO: 401 - RNA, 20 nt, Artificial sequence
  F12 RNAi agent antisense strand modified sequence
uuuguacuuaugcuccuugu

SEQ ID NO: 402 - RNA, 19 nt, Artificial sequence
  F12 RNAi agent antisense strand modified sequence
uuuguacuuaugcuccuug

SEQ ID NO: 403 - RNA, 21 nt, Artificial sequence
  F12 RNAi agent antisense strand modified sequence
auuguacuuaugcuccuuggg

SEQ ID NO: 404 - RNA, 21 nt, Artificial sequence
  F12 RNAi agent antisense strand modified sequence
uuuguacuuaugcuccuuggc

SEQ ID NO: 405 - RNA, 21 nt, Artificial sequence
  F12 RNAi agent antisense strand modified sequence
uuuguacuuaugcuccuuggc

SEQ ID NO: 406 - RNA, 21 nt, Artificial sequence
  F12 RNAi agent antisense strand modified sequence
uuguacuuaugcuccuugggc

SEQ ID NO: 407 - RNA, 21 nt, Artificial sequence
  F12 RNAi agent antisense strand modified sequence
uguacuuaugcuccuuggggc

SEQ ID NO: 408 - RNA, 21 nt, Artificial sequence
  F12 RNAi agent antisense strand modified sequence
uuuuguacuuaugcuccuugc

SEQ ID NO: 409 - RNA, 21 nt, Artificial sequence
  F12 RNAi agent antisense strand modified sequence
ucuuuguacuuaugcuccucg

SEQ ID NO: 410 - RNA, 21 nt, Artificial sequence
  F12 RNAi agent antisense strand modified sequence
ucuuuguacuuaugcuccucc

SEQ ID NO: 411 - RNA, 21 nt, Artificial sequence
  F12 RNAi agent antisense strand modified sequence
ucagcuuuguacuuaugcucc

SEQ ID NO: 412 - RNA, 21 nt, Artificial sequence
  F12 RNAi agent antisense strand modified sequence
ugguacauuugugguacagcu

SEQ ID NO: 413 - RNA, 21 nt, Artificial sequence
  F12 RNAi agent antisense strand modified sequence
uuuguacuuaugcuccuuggu

SEQ ID NO: 414 - RNA, 21 nt, Artificial sequence
  F12 RNAi agent antisense strand modified sequence
aucgaaaguguugacuccaag

SEQ ID NO: 415 - RNA, 21 nt, Artificial sequence
  F12 RNAi agent antisense strand modified sequence
aucgaaaguguugacuccagc

SEQ ID NO: 416 - RNA, 21 nt, Artificial sequence
  F12 RNAi agent antisense strand modified sequence
aaucgaaaguguugacuccac

SEQ ID NO: 417 - RNA, 21 nt, Artificial sequence
  F12 RNAi agent antisense strand modified sequence
uggaaucgaaaguguugacuc

SEQ ID NO: 418 - RNA, 21 nt, Artificial sequence
  F12 RNAi agent antisense strand modified sequence
uguacauuugugguacagcug

SEQ ID NO: 419 - RNA, 21 nt, Artificial sequence
  F12 RNAi agent antisense strand modified sequence
ucagcuuuguacuuaugcucg

SEQ ID NO: 420 - RNA, 21 nt, Artificial sequence
  F12 RNAi agent antisense strand modified sequence
ucagcuuuguacuuaugcucu

SEQ ID NO: 421 - RNA, 21 nt, Artificial sequence
  F12 RNAi agent antisense strand modified sequence
uuguacuuaugcuccuugggu

SEQ ID NO: 422 - RNA, 26 nt, Artificial sequence
  F12 RNAi agent sense strand modified sequence
uauaugcccaagaaagugaaagacca

SEQ ID NO: 423 - RNA, 26 nt, Artificial sequence
  F12 RNAi agent sense strand modified sequence
gcgagcccaagaaagugaaagaccaa

SEQ ID NO: 424 - RNA, 26 nt, Artificial sequence
  F12 RNAi agent sense strand modified sequence
gcgagcccaagaaagugaaagaccaa

SEQ ID NO: 425 - RNA, 26 nt, Artificial sequence
  F12 RNAi agent sense strand modified sequence
gcgagcccaagaaagugaaagaccaa

SEQ ID NO: 426 - RNA, 27 nt, Artificial sequence
  F12 RNAi agent sense strand modified sequence
gcgagcccaagaaagugaaagaccaaa

SEQ ID NO: 427 - RNA, 26 nt, Artificial sequence
  F12 RNAi agent sense strand modified sequence
gcguguuuggagcccaagaaagugaa

SEQ ID NO: 428 - RNA, 26 nt, Artificial sequence
  F12 RNAi agent sense strand modified sequence
gcgaugcccaagaaagugaaagacca

SEQ ID NO: 429 - RNA, 25 nt, Artificial sequence
  F12 RNAi agent sense strand modified sequence
gcgagcccaagaaagugaaagacca

SEQ ID NO: 430 - RNA, 25 nt, Artificial sequence
  F12 RNAi agent sense strand modified sequence
gcguguuuggagcccaagaaaguga

SEQ ID NO: 431 - RNA, 26 nt, Artificial sequence
  F12 RNAi agent sense strand modified sequence
gcgaugcccaagaaagugaaagacca

SEQ ID NO: 432 - DNA, 26 bp, Artificial sequence
  F12 RNAi agent sense strand modified sequence
gcgaugcccaagaaagugaaagacct

SEQ ID NO: 433 - RNA, 26 nt, Artificial sequence
  F12 RNAi agent sense strand modified sequence
gcgaugcccaagaaagugaaagacca

SEQ ID NO: 434 - RNA, 26 nt, Artificial sequence
  F12 RNAi agent sense strand modified sequence
gcgaugcccaagaaagugaaagacca

SEQ ID NO: 435 - RNA, 26 nt, Artificial sequence
  F12 RNAi agent sense strand modified sequence
gcgaugcccaagaaagugaaagacca

SEQ ID NO: 436 - RNA, 25 nt, Artificial sequence
  F12 RNAi agent sense strand modified sequence
gcgaugcccaagaaagugaaagacc

SEQ ID NO: 437 - RNA, 26 nt, Artificial sequence
  F12 RNAi agent sense strand modified sequence
gcgaugcccaagaaagugaaagacca

SEQ ID NO: 438 - RNA, 26 nt, Artificial sequence
  F12 RNAi agent sense strand modified sequence
gcgaugcccaagaaagugaaagacca

SEQ ID NO: 439 - RNA, 26 nt, Artificial sequence
  F12 RNAi agent sense strand modified sequence
ugauuggagcccaagaaagugaaaga

SEQ ID NO: 440 - RNA, 21 nt, Artificial sequence
  F12 RNAi agent sense strand modified sequence
agcccaagaaagugaaagauu

SEQ ID NO: 441 - RNA, 25 nt, Artificial sequence
  F12 RNAi agent sense strand modified sequence
aaggagcccaagaaagugaaagauu

SEQ ID NO: 442 - RNA, 26 nt, Artificial sequence
  F12 RNAi agent sense strand modified sequence
ugaggagcccaagaaagugaaagaca

SEQ ID NO: 443 - RNA, 21 nt, Artificial sequence
  F12 RNAi agent sense strand modified sequence
cccaagaaagugaaagacauu

SEQ ID NO: 444 - RNA, 25 nt, Artificial sequence
  F12 RNAi agent sense strand modified sequence
aaagcccaagaaagugaaagacauu

SEQ ID NO: 445 - RNA, 26 nt, Artificial sequence
  F12 RNAi agent sense strand modified sequence
ugaagcccaagaaagugaaagaccaa

SEQ ID NO: 446 - RNA, 21 nt, Artificial sequence
  F12 RNAi agent sense strand modified sequence
caagaaagugaaagaccaauu

SEQ ID NO: 447 - RNA, 25 nt, Artificial sequence
  F12 RNAi agent sense strand modified sequence
aacccaagaaagugaaagaccaauu

SEQ ID NO: 448 - RNA, 26 nt, Artificial sequence
  F12 RNAi agent sense strand modified sequence
ugaaagugcuuugagccucagcuuca

SEQ ID NO: 449 - RNA, 21 nt, Artificial sequence
  F12 RNAi agent sense strand modified sequence
gcuuugagccucagcuucauu

SEQ ID NO: 450 - RNA, 25 nt, Artificial sequence
  F12 RNAi agent sense strand modified sequence
aagugcuuugagccucagcuucauu

SEQ ID NO: 451 - RNA, 26 nt, Artificial sequence
  F12 RNAi agent sense strand modified sequence
ugagugcuuugagccucagcuucuca

SEQ ID NO: 452 - RNA, 21 nt, Artificial sequence
  F12 RNAi agent sense strand modified sequence
uuugagccucagcuucucauu

SEQ ID NO: 453 - RNA, 25 nt, Artificial sequence
  F12 RNAi agent sense strand modified sequence
aagcuuugagccucagcuucucauu

SEQ ID NO: 454 - RNA, 26 nt, Artificial sequence
  F12 RNAi agent sense strand modified sequence
ugaacucaauaaagugcuuugaaaaa

SEQ ID NO: 455 - RNA, 21 nt, Artificial sequence
  F12 RNAi agent sense strand modified sequence
aauaaagugcuuugaaaaauu

SEQ ID NO: 456 - RNA, 25 nt, Artificial sequence
  F12 RNAi agent sense strand modified sequence
aaucaauaaagugcuuugaaaaauu

SEQ ID NO: 457 - RNA, 26 nt, Artificial sequence
  F12 RNAi agent sense strand modified sequence
ugaaugcccaagaaagugaaagacca

SEQ ID NO: 458 - RNA, 21 nt, Artificial sequence
  F12 RNAi agent sense strand modified sequence
ccaagaaagugaaagaccauu

SEQ ID NO: 459 - RNA, 25 nt, Artificial sequence
  F12 RNAi agent sense strand modified sequence
aagcccaagaaagugaaagaccauu

SEQ ID NO: 460 - RNA, 26 nt, Artificial sequence
  F12 RNAi agent sense strand modified sequence
ugaaugcccaagaaagugaaagacca

SEQ ID NO: 461 - RNA, 26 nt, Artificial sequence
  F12 RNAi agent sense strand modified sequence
ugaaugcccaagaaagugaaagacca

SEQ ID NO: 462 - RNA, 26 nt, Artificial sequence
  F12 RNAi agent sense strand modified sequence
ugaaugcccaagaaagugaaagacca

SEQ ID NO: 463 - RNA, 26 nt, Artificial sequence
  F12 RNAi agent sense strand modified sequence
ugaaugcccaagaaagugaaagacca

SEQ ID NO: 464 - RNA, 26 nt, Artificial sequence
  F12 RNAi agent sense strand modified sequence
uauaugcccaagaaagugaaagacca

SEQ ID NO: 465 - RNA, 26 nt, Artificial sequence
  F12 RNAi agent sense strand modified sequence
ugaaugcccaagaaagugaaagacca

SEQ ID NO: 466 - RNA, 26 nt, Artificial sequence
  F12 RNAi agent sense strand modified sequence
ugagugcccaagaaagugaaagacca

SEQ ID NO: 467 - RNA, 26 nt, Artificial sequence
  F12 RNAi agent sense strand modified sequence
gcggagcccaagaaagugaaagacca

SEQ ID NO: 468 - RNA, 26 nt, Artificial sequence
  F12 RNAi agent sense strand modified sequence
ugagugcccaagaaagugaaagacca

SEQ ID NO: 469 - RNA, 26 nt, Artificial sequence
  F12 RNAi agent sense strand modified sequence
gcggagcccaagaaagugaaagacca

SEQ ID NO: 470 - RNA, 26 nt, Artificial sequence
  F12 RNAi agent sense strand modified sequence
uauaugcccaagaaagugaaagacca

SEQ ID NO: 471 - RNA, 26 nt, Artificial sequence
  F12 RNAi agent sense strand modified sequence
uuggugcccaagaaagugaaagacca

SEQ ID NO: 472 - RNA, 26 nt, Artificial sequence
  F12 RNAi agent sense strand modified sequence
aaggugcccaagaaagugaaagacca

SEQ ID NO: 473 - RNA, 26 nt, Artificial sequence
  F12 RNAi agent sense strand modified sequence
guggugcccaagaaagugaaagacca

SEQ ID NO: 474 - RNA, 26 nt, Artificial sequence
  F12 RNAi agent sense strand modified sequence
gaggugcccaagaaagugaaagacca

SEQ ID NO: 475 - RNA, 25 nt, Artificial sequence
  F12 RNAi agent sense strand modified sequence
aagcccaagaaagugaaagaccauu

SEQ ID NO: 476 - RNA, 25 nt, Artificial sequence
  F12 RNAi agent sense strand modified sequence
aagcccaagaaagugaaagaccauu

SEQ ID NO: 477 - RNA, 25 nt, Artificial sequence
  F12 RNAi agent sense strand modified sequence
aagcccaagaaagugaaagaccauu

SEQ ID NO: 478 - RNA, 23 nt, Artificial sequence
  F12 RNAi agent sense strand modified sequence
aagcccaagaaagugaaagacca

SEQ ID NO: 479 - RNA, 23 nt, Artificial sequence
  F12 RNAi agent sense strand modified sequence
aagcccaagaaagugaaagacca

SEQ ID NO: 480 - RNA, 23 nt, Artificial sequence
  F12 RNAi agent sense strand modified sequence
aagcccaagaaagugaaagacca

SEQ ID NO: 481 - RNA, 23 nt, Artificial sequence
  F12 RNAi agent sense strand modified sequence
aagcccaagaaagugaaagacca

SEQ ID NO: 482 - RNA, 25 nt, Artificial sequence
  F12 RNAi agent sense strand modified sequence
aagcccaagaaagugaaagaccauu

SEQ ID NO: 483 - RNA, 23 nt, Artificial sequence
  F12 RNAi agent sense strand modified sequence
aagcccaagaaagugaaagacca

SEQ ID NO: 484 - RNA, 23 nt, Artificial sequence
  F12 RNAi agent sense strand modified sequence
aagcccaagaaagugaaagacca

SEQ ID NO: 485 - RNA, 21 nt, Artificial sequence
  F12 RNAi agent sense strand modified sequence
ccaagaaagugaaagaccauu

SEQ ID NO: 486 - RNA, 25 nt, Artificial sequence
  F12 RNAi agent sense strand modified sequence
aagcccaagaaagugaaagaccauu

SEQ ID NO: 487 - RNA, 26 nt, Artificial sequence
  F12 RNAi agent sense strand modified sequence
ugauuggagcccaagaaagugaaaga

SEQ ID NO: 488 - RNA, 26 nt, Artificial sequence
  F12 RNAi agent sense strand modified sequence
ugaggagcccaagaaagugaaagaca

SEQ ID NO: 489 - RNA, 26 nt, Artificial sequence
  F12 RNAi agent sense strand modified sequence
ugaagcccaagaaagugaaagaccaa

SEQ ID NO: 490 - RNA, 26 nt, Artificial sequence
  F12 RNAi agent sense strand modified sequence
ugaaagugcuuugagccucagcuuca

SEQ ID NO: 491 - RNA, 26 nt, Artificial sequence
  F12 RNAi agent sense strand modified sequence
ugagugcuuugagccucagcuucuca

SEQ ID NO: 492 - RNA, 26 nt, Artificial sequence
  F12 RNAi agent sense strand modified sequence
ugaacucaauaaagugcuuugaaaaa

SEQ ID NO: 493 - RNA, 26 nt, Artificial sequence
  F12 RNAi agent sense strand modified sequence
ugaaugcccaagaaagugaaagacca

SEQ ID NO: 494 - RNA, 26 nt, Artificial sequence
  F12 RNAi agent sense strand modified sequence
ugaaugcccaagaaagugaaagacca

SEQ ID NO: 495 - RNA, 25 nt, Artificial sequence
  F12 RNAi agent sense strand modified sequence
aagcccaagaaagugaaagaccauu

SEQ ID NO: 496 - RNA, 25 nt, Artificial sequence
  F12 RNAi agent sense strand modified sequence
aagcccaagaaagugaaagaccauu

SEQ ID NO: 497 - RNA, 25 nt, Artificial sequence
  F12 RNAi agent sense strand modified sequence
aagcccaagaaagugaaagaccauu

SEQ ID NO: 498 - RNA, 21 nt, Artificial sequence
  F12 RNAi agent sense strand modified sequence
acacaagaaagugaaagacca

SEQ ID NO: 499 - RNA, 21 nt, Artificial sequence
  F12 RNAi agent sense strand modified sequence
gcccaagaaagugaaagacca

SEQ ID NO: 500 - RNA, 26 nt, Artificial sequence
  F12 RNAi agent sense strand modified sequence
gcggagcccaagaaagugaaagacca

SEQ ID NO: 501 - RNA, 23 nt, Artificial sequence
  F12 RNAi agent sense strand modified sequence
aagcccaagaaagugaaagacca

SEQ ID NO: 502 - RNA, 23 nt, Artificial sequence
  F12 RNAi agent sense strand modified sequence
gagcccaagaaagugaaagacca

SEQ ID NO: 503 - RNA, 21 nt, Artificial sequence
  F12 RNAi agent sense strand modified sequence
gcccaagaaagugaaagacca

SEQ ID NO: 504 - RNA, 21 nt, Artificial sequence
  F12 RNAi agent sense strand modified sequence
aaccaagaaagugaaagacca

SEQ ID NO: 505 - RNA, 23 nt, Artificial sequence
  F12 RNAi agent sense strand modified sequence
aagcccaagaaagugaaagacca

SEQ ID NO: 506 - DNA, 26 bp, Artificial sequence
  F12 RNAi agent sense strand modified sequence
ugaacucaauaaagugcuuugaaaat

SEQ ID NO: 507 - RNA, 22 nt, Artificial sequence
  F12 RNAi agent sense strand modified sequence
cucaauaaagugcuuugaaaaa

SEQ ID NO: 508 - RNA, 22 nt, Artificial sequence
  F12 RNAi agent sense strand modified sequence
cucaauaaagugcuuugaaaaa

SEQ ID NO: 509 - RNA, 22 nt, Artificial sequence
  F12 RNAi agent sense strand modified sequence
aucaauaaagugcuuugaaaaa

SEQ ID NO: 510 - RNA, 21 nt, Artificial sequence
  F12 RNAi agent sense strand modified sequence
ucaauaaagugcuuugaaaaa

SEQ ID NO: 511 - RNA, 21 nt, Artificial sequence
  F12 RNAi agent sense strand modified sequence
gcaauaaagugcuuugaaaaa

SEQ ID NO: 512 - RNA, 21 nt, Artificial sequence
  F12 RNAi agent sense strand modified sequence
ucgauaaagugcuuugaaaaa

SEQ ID NO: 513 - RNA, 19 nt, Artificial sequence
  F12 RNAi agent sense strand modified sequence
gcuuugagccucagcuuca

SEQ ID NO: 514 - RNA, 19 nt, Artificial sequence
  F12 RNAi agent sense strand modified sequence
gcuuugagccucagcuuca

SEQ ID NO: 515 - RNA, 21 nt, Artificial sequence
  F12 RNAi agent sense strand modified sequence
aagcuuugagccucagcuuca

SEQ ID NO: 516 - RNA, 21 nt, Artificial sequence
  F12 RNAi agent sense strand modified sequence
aagcuuugagccucagcuuca

SEQ ID NO: 517 - RNA, 21 nt, Artificial sequence
  F12 RNAi agent sense strand modified sequence
aagcuuugagccucagcuuca

SEQ ID NO: 518 - RNA, 21 nt, Artificial sequence
  F12 RNAi agent sense strand modified sequence
gugcuuugagccucagcuuca

SEQ ID NO: 519 - RNA, 21 nt, Artificial sequence
  F12 RNAi agent sense strand modified sequence
aggaacucaauaaagugcuua

SEQ ID NO: 520 - RNA, 20 nt, Artificial sequence
  F12 RNAi agent sense strand modified sequence
ggaacucaauaaagugcuua

SEQ ID NO: 521 - RNA, 21 nt, Artificial sequence
  F12 RNAi agent sense strand modified sequence
gaacucaauaaagugcuuuga

SEQ ID NO: 522 - RNA, 22 nt, Artificial sequence
  F12 RNAi agent sense strand modified sequence
agaacucaauaaagugcuuuga

SEQ ID NO: 523 - RNA, 21 nt, Artificial sequence
  F12 RNAi agent sense strand modified sequence
aacucaauaaagugcugugaa

SEQ ID NO: 524 - RNA, 22 nt, Artificial sequence
  F12 RNAi agent sense strand modified sequence
gaacucaauaaagugcuuugaa

SEQ ID NO: 525 - RNA, 23 nt, Artificial sequence
  F12 RNAi agent sense strand modified sequence
agaacucaauaaagugcuuugaa

SEQ ID NO: 526 - RNA, 21 nt, Artificial sequence
  F12 RNAi agent sense strand modified sequence
acucaauaaagugcuuugaaa

SEQ ID NO: 527 - RNA, 21 nt, Artificial sequence
  F12 RNAi agent sense strand modified sequence
acucaauaaagugcuuugaau

SEQ ID NO: 528 - RNA, 23 nt, Artificial sequence
  F12 RNAi agent sense strand modified sequence
gaacucaauaaagugcuuugaaa

SEQ ID NO: 529 - RNA, 21 nt, Artificial sequence
  F12 RNAi agent sense strand modified sequence
aggaacucaauaaagugcuua

SEQ ID NO: 530 - RNA, 21 nt, Artificial sequence
  F12 RNAi agent sense strand modified sequence
gaacucaauaaagugcuuuga

SEQ ID NO: 531 - RNA, 21 nt, Artificial sequence
  F12 RNAi agent sense strand modified sequence
aacucaauaaagugcugugaa

SEQ ID NO: 532 - RNA, 21 nt, Artificial sequence
  F12 RNAi agent sense strand modified sequence
acucaauaaagugcuuugaaa

SEQ ID NO: 533 - RNA, 21 nt, Artificial sequence
  F12 RNAi agent sense strand modified sequence
acaauaaagugcuuugaaaaa

SEQ ID NO: 534 - RNA, 21 nt, Artificial sequence
  F12 RNAi agent sense strand modified sequence
acaauaaagugcuuugaaaaa

SEQ ID NO: 535 - RNA, 28 nt, Artificial sequence
  F12 RNAi agent sense strand modified sequence
ugaacucaauaaagugcuuugaaaaauu

SEQ ID NO: 536 - RNA, 21 nt, Artificial sequence
  F12 RNAi agent sense strand modified sequence
acaauaaagugcuuugaaaaa

SEQ ID NO: 537 - RNA, 23 nt, Artificial sequence
  F12 RNAi agent sense strand modified sequence
acaauaaagugcuuugaaaaauu

SEQ ID NO: 538 - RNA, 23 nt, Artificial sequence
  F12 RNAi agent sense strand modified sequence
aggaacucaauaaagugcuuauu

SEQ ID NO: 539 - RNA, 23 nt, Artificial sequence
  F12 RNAi agent sense strand modified sequence
aacucaauaaagugcuuugaauu

SEQ ID NO: 540 - RNA, 23 nt, Artificial sequence
  F12 RNAi agent sense strand modified sequence
aagcccaagaaagugaaagacca

SEQ ID NO: 541 - RNA, 21 nt, Artificial sequence
  F12 RNAi agent sense strand modified sequence
gcccaagaaagugaaagacca

SEQ ID NO: 542 - RNA, 21 nt, Artificial sequence
  F12 RNAi agent sense strand modified sequence
aaccaagaaagugaaagacca

SEQ ID NO: 543 - RNA, 22 nt, Artificial sequence
  F12 RNAi agent sense strand modified sequence
cucaauaaagugcuuugaaaaa

SEQ ID NO: 544 - RNA, 22 nt, Artificial sequence
  F12 RNAi agent sense strand modified sequence
cucaauaaagugcuuugaaaaa

SEQ ID NO: 545 - RNA, 22 nt, Artificial sequence
  F12 RNAi agent sense strand modified sequence
aucaauaaagugcuuugaaaaa

SEQ ID NO: 546 - RNA, 21 nt, Artificial sequence
  F12 RNAi agent sense strand modified sequence
ucaauaaagugcuuugaaaaa

SEQ ID NO: 547 - RNA, 21 nt, Artificial sequence
  F12 RNAi agent sense strand modified sequence
gcaauaaagugcuuugaaaaa

SEQ ID NO: 548 - RNA, 21 nt, Artificial sequence
  F12 RNAi agent sense strand modified sequence
ucgauaaagugcuuugaaaaa

SEQ ID NO: 549 - RNA, 21 nt, Artificial sequence
  F12 RNAi agent sense strand modified sequence
gcccaagaaagugaaagacca

SEQ ID NO: 550 - RNA, 21 nt, Artificial sequence
  F12 RNAi agent sense strand modified sequence
gcccaagaaagugaaagacca

SEQ ID NO: 551 - RNA, 21 nt, Artificial sequence
  F12 RNAi agent sense strand modified sequence
gcccaagaaagugaaagacca

SEQ ID NO: 552 - RNA, 21 nt, Artificial sequence
  F12 RNAi agent sense strand modified sequence
aaccaagaaagugaaagacca

SEQ ID NO: 553 - RNA, 21 nt, Artificial sequence
  F12 RNAi agent sense strand modified sequence
aaccaagaaagugaaagacca

SEQ ID NO: 554 - RNA, 21 nt, Artificial sequence
  F12 RNAi agent sense strand modified sequence
aaccaagaaagugaaagacca

SEQ ID NO: 555 - RNA, 21 nt, Artificial sequence
  F12 RNAi agent sense strand modified sequence
gaccaagaaagugaaagacca

SEQ ID NO: 556 - RNA, 21 nt, Artificial sequence
  F12 RNAi agent sense strand modified sequence
gcucaauaaagugcuuugaaa

SEQ ID NO: 557 - RNA, 21 nt, Artificial sequence
  F12 RNAi agent sense strand modified sequence
gacucaauaaagugcuuugaa

SEQ ID NO: 558 - RNA, 21 nt, Artificial sequence
  F12 RNAi agent sense strand modified sequence
agcucaauaaagugcuuugaa

SEQ ID NO: 559 - RNA, 21 nt, Artificial sequence
  F12 RNAi agent sense strand modified sequence
ggcucaauaaagugcuuugaa

SEQ ID NO: 560 - RNA, 22 nt, Artificial sequence
  F12 RNAi agent sense strand modified sequence
ggacucaauaaagugcuuugaa

SEQ ID NO: 561 - RNA, 19 nt, Artificial sequence
  F12 RNAi agent sense strand modified sequence
cucaauaaagugcuuugaa

SEQ ID NO: 562 - RNA, 21 nt, Artificial sequence
  F12 RNAi agent sense strand modified sequence
cucaauaaagugcuuugaauu

SEQ ID NO: 563 - RNA, 21 nt, Artificial sequence
  F12 RNAi agent sense strand modified sequence
cucaauaaagugcuuugaauu

SEQ ID NO: 564 - RNA, 22 nt, Artificial sequence
  F12 RNAi agent sense strand modified sequence
aacucaauaaagugcuuugaaa

SEQ ID NO: 565 - RNA, 22 nt, Artificial sequence
  F12 RNAi agent sense strand modified sequence
agcucaauaaagugcuuugaaa

SEQ ID NO: 566 - RNA, 22 nt, Artificial sequence
  F12 RNAi agent sense strand modified sequence
gacucaauaaagugcuuugaaa

SEQ ID NO: 567 - RNA, 23 nt, Artificial sequence
  F12 RNAi agent sense strand modified sequence
ggacucaauaaagugcuuugaaa

SEQ ID NO: 568 - RNA, 19 nt, Artificial sequence
  F12 RNAi agent sense strand modified sequence
ucaauaaagugcuuugaaa

SEQ ID NO: 569 - RNA, 21 nt, Artificial sequence
  F12 RNAi agent sense strand modified sequence
ucaauaaagugcuuugaaauu

SEQ ID NO: 570 - RNA, 22 nt, Artificial sequence
  F12 RNAi agent sense strand modified sequence
ggcucaauaaagugcuuugaaa

SEQ ID NO: 571 - RNA, 21 nt, Artificial sequence
  F12 RNAi agent sense strand modified sequence
ucaauaaagugcuuugaaauu

SEQ ID NO: 572 - RNA, 21 nt, Artificial sequence
  F12 RNAi agent sense strand modified sequence
ucaauaaagugcuuugaaauu

SEQ ID NO: 573 - RNA, 21 nt, Artificial sequence
  F12 RNAi agent sense strand modified sequence
ucaauaaagugcuuugaaauu

SEQ ID NO: 574 - RNA, 21 nt, Artificial sequence
  F12 RNAi agent sense strand modified sequence
acucaauaaagugcuuugaaa

SEQ ID NO: 575 - RNA, 23 nt, Artificial sequence
  F12 RNAi agent sense strand modified sequence
gaacucaauaaagugcuuugaaa

SEQ ID NO: 576 - RNA, 21 nt, Artificial sequence
  F12 RNAi agent sense strand modified sequence
acucaauaaagugcuuugaaa

SEQ ID NO: 577 - RNA, 21 nt, Artificial sequence
  F12 RNAi agent sense strand modified sequence
acucaauaaagugcuuugaaa

SEQ ID NO: 578 - RNA, 21 nt, Artificial sequence
  F12 RNAi agent sense strand modified sequence
gggaacucaauaaagugcuua

SEQ ID NO: 579 - RNA, 21 nt, Artificial sequence
  F12 RNAi agent sense strand modified sequence
aggaacucaauaaagugcuuu

SEQ ID NO: 580 - RNA, 22 nt, Artificial sequence
  F12 RNAi agent sense strand modified sequence
caggaacucaauaaagugcuua

SEQ ID NO: 581 - RNA, 21 nt, Artificial sequence
  F12 RNAi agent sense strand modified sequence
gaacucaauaaagugcuuauu

SEQ ID NO: 582 - RNA, 21 nt, Artificial sequence
  F12 RNAi agent sense strand modified sequence
gaacucaauaaagugcuuauu

SEQ ID NO: 583 - RNA, 21 nt, Artificial sequence
  F12 RNAi agent sense strand modified sequence
gaacucaauaaagugcuuauu

SEQ ID NO: 584 - RNA, 21 nt, Artificial sequence
  F12 RNAi agent sense strand modified sequence
aggaacucaauaaagugcuua

SEQ ID NO: 585 - RNA, 21 nt, Artificial sequence
  F12 RNAi agent sense strand modified sequence
aggaacucaauaaagugcuua

SEQ ID NO: 586 - RNA, 21 nt, Artificial sequence
  F12 RNAi agent sense strand modified sequence
aggaacucaauaaagugcuua

SEQ ID NO: 587 - RNA, 21 nt, Artificial sequence
  F12 RNAi agent sense strand modified sequence
aggaacucaauaaagugcuua

SEQ ID NO: 588 - RNA, 21 nt, Artificial sequence
  F12 RNAi agent sense strand modified sequence
aggaacucaauaaagugcuua

SEQ ID NO: 589 - RNA, 21 nt, Artificial sequence
  F12 RNAi agent sense strand modified sequence
aacucaauaaagugcugugaa

SEQ ID NO: 590 - RNA, 21 nt, Artificial sequence
  F12 RNAi agent sense strand modified sequence
aacucaauaaagugcugugaa

SEQ ID NO: 591 - RNA, 22 nt, Artificial sequence
  F12 RNAi agent sense strand modified sequence
gaacucaauaaagugcugugaa

SEQ ID NO: 592 - RNA, 22 nt, Artificial sequence
  F12 RNAi agent sense strand modified sequence
gaacucaauaaagugcugugaa

SEQ ID NO: 593 - RNA, 21 nt, Artificial sequence
  F12 RNAi agent sense strand modified sequence
aacucaauaaagugcugugaa

SEQ ID NO: 594 - RNA, 22 nt, Artificial sequence
  F12 RNAi agent sense strand modified sequence
gaacucaauaaagugcugugaa

SEQ ID NO: 595 - RNA, 21 nt, Artificial sequence
  F12 RNAi agent sense strand modified sequence
gcccaagaaagugaaagacca

SEQ ID NO: 596 - RNA, 21 nt, Artificial sequence
  F12 RNAi agent sense strand modified sequence
gcccaagaaagugaaagacca

SEQ ID NO: 597 - RNA, 21 nt, Artificial sequence
  F12 RNAi agent sense strand modified sequence
aacucaauaaagugcugugaa

SEQ ID NO: 598 - RNA, 21 nt, Artificial sequence
  F12 RNAi agent sense strand modified sequence
aacucaauaaagugcugugaa

SEQ ID NO: 599 - RNA, 21 nt, Artificial sequence
  F12 RNAi agent sense strand modified sequence
aacucaauaaagugcugugaa

SEQ ID NO: 600 - RNA, 21 nt, Artificial sequence
  F12 RNAi agent sense strand modified sequence
uuggagcccaagaaagugaaa

SEQ ID NO: 601 - RNA, 21 nt, Artificial sequence
  F12 RNAi agent sense strand modified sequence
uuggagcccaagaaagugaaa

SEQ ID NO: 602 - RNA, 21 nt, Artificial sequence
  F12 RNAi agent sense strand modified sequence
uuggagcccaagaaagugaaa

SEQ ID NO: 603 - RNA, 19 nt, Artificial sequence
  F12 RNAi agent sense strand modified sequence
ggagcccaagaaagugaaa

SEQ ID NO: 604 - RNA, 21 nt, Artificial sequence
  F12 RNAi agent sense strand modified sequence
ggagcccaagaaagugaaauu

SEQ ID NO: 605 - RNA, 21 nt, Artificial sequence
  F12 RNAi agent sense strand modified sequence
ggagcccaagaaagugaaauu

SEQ ID NO: 606 - RNA, 21 nt, Artificial sequence
  F12 RNAi agent sense strand modified sequence
cccaaggagcauaaguacaaa

SEQ ID NO: 607 - RNA, 21 nt, Artificial sequence
  F12 RNAi agent sense strand modified sequence
uuggagucaacacuuucgaua

SEQ ID NO: 608 - RNA, 21 nt, Artificial sequence
  F12 RNAi agent sense strand modified sequence
ccaaggagcauaaguacaauu

SEQ ID NO: 609 - RNA, 21 nt, Artificial sequence
  F12 RNAi agent sense strand modified sequence
cgcaagagucugucuucgauu

SEQ ID NO: 610 - RNA, 21 nt, Artificial sequence
  F12 RNAi agent sense strand modified sequence
aacucaauaaagugcuuugaa

SEQ ID NO: 611 - RNA, 21 nt, Artificial sequence
  F12 RNAi agent sense strand modified sequence
cccaaggagcauaaguacaaa

SEQ ID NO: 612 - RNA, 21 nt, Artificial sequence
  F12 RNAi agent sense strand modified sequence
uuggagucaacacuuucgaua

SEQ ID NO: 613 - RNA, 21 nt, Artificial sequence
  F12 RNAi agent sense strand modified sequence
ccaaggagcauaaguacaauu

SEQ ID NO: 614 - RNA, 21 nt, Artificial sequence
  F12 RNAi agent sense strand modified sequence
cgcaagagucugucuucgauu

SEQ ID NO: 615 - RNA, 21 nt, Artificial sequence
  F12 RNAi agent sense strand modified sequence
aacucaauaaagugcugugaa

SEQ ID NO: 616 - RNA, 21 nt, Artificial sequence
  F12 RNAi agent sense strand modified sequence
aacucaauaaagugcuuugaa

SEQ ID NO: 617 - RNA, 23 nt, Artificial sequence
  F12 RNAi agent sense strand modified sequence
ggaacucaauaaagugcuuugaa

SEQ ID NO: 618 - RNA, 22 nt, Artificial sequence
  F12 RNAi agent sense strand modified sequence
gaacucaauaaagugcugugaa

SEQ ID NO: 619 - RNA, 24 nt, Artificial sequence
  F12 RNAi agent sense strand modified sequence
gaacucaauaaagugcuuugaauu

SEQ ID NO: 620 - RNA, 21 nt, Artificial sequence
  F12 RNAi agent sense strand modified sequence
cucaauaaagugcuuugaauu

SEQ ID NO: 621 - RNA, 22 nt, Artificial sequence
  F12 RNAi agent sense strand modified sequence
ggaacucaauaaagugcuuuga

SEQ ID NO: 622 - RNA, 21 nt, Artificial sequence
  F12 RNAi agent sense strand modified sequence
ggagucaacacuuucgauauu

SEQ ID NO: 623 - RNA, 19 nt, Artificial sequence
  F12 RNAi agent sense strand modified sequence
ggagucaacacuuucgaua

SEQ ID NO: 624 - RNA, 22 nt, Artificial sequence
  F12 RNAi agent sense strand modified sequence
cuuggagucaacacuuucgaua

SEQ ID NO: 625 - RNA, 21 nt, Artificial sequence
  F12 RNAi agent sense strand modified sequence
ccccaaggagcauaaguacaa

SEQ ID NO: 626 - RNA, 21 nt, Artificial sequence
  F12 RNAi agent sense strand modified sequence
caaggagcauaaguacaaauu

SEQ ID NO: 627 - RNA, 21 nt, Artificial sequence
  F12 RNAi agent sense strand modified sequence
cccaaggagcauaaguacaaa

SEQ ID NO: 628 - RNA, 22 nt, Artificial sequence
  F12 RNAi agent sense strand modified sequence
ccccaaggagcauaaguacaaa

SEQ ID NO: 629 - RNA, 23 nt, Artificial sequence
  F12 RNAi agent sense strand modified sequence
cccaaggagcauaaguacaaauu

SEQ ID NO: 630 - RNA, 21 nt, Artificial sequence
  F12 RNAi agent sense strand modified sequence
ccccaaggagcauaaguacaa

SEQ ID NO: 631 - RNA, 22 nt, Artificial sequence
  F12 RNAi agent sense strand modified sequence
cccaaggagcauaaguacaauu

SEQ ID NO: 632 - RNA, 22 nt, Artificial sequence
  F12 RNAi agent sense strand modified sequence
cuuggagucaacacuuucgaua

SEQ ID NO: 633 - RNA, 23 nt, Artificial sequence
  F12 RNAi agent sense strand modified sequence
gcuuggagucaacacuuucgaua

SEQ ID NO: 634 - RNA, 21 nt, Artificial sequence
  F12 RNAi agent sense strand modified sequence
cccaaggagcauaaguacaaa

SEQ ID NO: 635 - RNA, 21 nt, Artificial sequence
  F12 RNAi agent sense strand modified sequence
cccaaggagcauaaguacaaa

SEQ ID NO: 636 - RNA, 21 nt, Artificial sequence
  F12 RNAi agent sense strand modified sequence
cccaaggagcauaaguacaaa

SEQ ID NO: 637 - RNA, 20 nt, Artificial sequence
  F12 RNAi agent sense strand modified sequence
ccaaggagcauaaguacaaa

SEQ ID NO: 638 - RNA, 19 nt, Artificial sequence
  F12 RNAi agent sense strand modified sequence
caaggagcauaaguacaaa

SEQ ID NO: 639 - RNA, 21 nt, Artificial sequence
  F12 RNAi agent sense strand modified sequence
cccaaggagcauaaguacaau

SEQ ID NO: 640 - RNA, 21 nt, Artificial sequence
  F12 RNAi agent sense strand modified sequence
acucaauaaagugcuuugaaa

SEQ ID NO: 641 - RNA, 21 nt, Artificial sequence
  F12 RNAi agent sense strand modified sequence
gccaaggagcauaaguacaaa

SEQ ID NO: 642 - RNA, 21 nt, Artificial sequence
  F12 RNAi agent sense strand modified sequence
  modified_base 15: n = i (inosine)
gccaaggagcauaanuacaaa

SEQ ID NO: 643 - RNA, 21 nt, Artificial sequence
  F12 RNAi agent sense strand modified sequence
gccaaggagcauaaguacaaa

SEQ ID NO: 644 - RNA, 21 nt, Artificial sequence
  F12 RNAi agent sense strand modified sequence
gcccaaggagcauaaguacaa

SEQ ID NO: 645 - RNA, 21 nt, Artificial sequence
  F12 RNAi agent sense strand modified sequence
gccccaaggagcauaaguaca

SEQ ID NO: 646 - RNA, 21 nt, Artificial sequence
  F12 RNAi agent sense strand modified sequence
gcaaggagcauaaguacaaaa

SEQ ID NO: 647 - RNA, 21 nt, Artificial sequence
  F12 RNAi agent sense strand modified sequence
cgaggagcauaaguacaaaga

SEQ ID NO: 648 - RNA, 21 nt, Artificial sequence
  F12 RNAi agent sense strand modified sequence
ggaggagcauaaguacaaaga

SEQ ID NO: 649 - RNA, 21 nt, Artificial sequence
  F12 RNAi agent sense strand modified sequence
ggagcauaaguacaaagcuga

SEQ ID NO: 650 - RNA, 21 nt, Artificial sequence
  F12 RNAi agent sense strand modified sequence
agcuguaccacaaauguacca

SEQ ID NO: 651 - RNA, 21 nt, Artificial sequence
  F12 RNAi agent sense strand modified sequence
accaaggagcauaaguacaaa

SEQ ID NO: 652 - RNA, 21 nt, Artificial sequence
  F12 RNAi agent sense strand modified sequence
accaaggagcauaaguacaaa

SEQ ID NO: 653 - RNA, 21 nt, Artificial sequence
  F12 RNAi agent sense strand modified sequence
gccaaggagcauaaguacaaa

SEQ ID NO: 654 - RNA, 21 nt, Artificial sequence
  F12 RNAi agent sense strand modified sequence
cuuggagucaacacuuucgau

SEQ ID NO: 655 - RNA, 21 nt, Artificial sequence
  F12 RNAi agent sense strand modified sequence
gcuggagucaacacuuucgau

SEQ ID NO: 656 - RNA, 21 nt, Artificial sequence
  F12 RNAi agent sense strand modified sequence
guggagucaacacuuucgauu

SEQ ID NO: 657 - RNA, 21 nt, Artificial sequence
  F12 RNAi agent sense strand modified sequence
gagucaacacuuucgauucca

SEQ ID NO: 658 - RNA, 21 nt, Artificial sequence
  F12 RNAi agent sense strand modified sequence
cagcuguaccacaaauguaca

SEQ ID NO: 659 - RNA, 21 nt, Artificial sequence
  F12 RNAi agent sense strand modified sequence
cgagcauaaguacaaagcuga

SEQ ID NO: 660 - RNA, 21 nt, Artificial sequence
  F12 RNAi agent sense strand modified sequence
agagcauaaguacaaagcuga

SEQ ID NO: 661 - RNA, 21 nt, Artificial sequence
  F12 RNAi agent sense strand modified sequence
acccaaggagcauaaguacaa

SEQ ID NO: 662 - RNA, 21 nt, Artificial sequence
  F12 RNAi agent antisense strand base sequence
aaagcacuuuauugaguuccu

SEQ ID NO: 663 - RNA, 21 nt, Artificial sequence
  F12 RNAi agent antisense strand base sequence
aaucgaaaguguugacuccac

SEQ ID NO: 664 - RNA, 21 nt, Artificial sequence
  F12 RNAi agent antisense strand base sequence
aggucuuucacuuucaugggu

SEQ ID NO: 665 - RNA, 21 nt, Artificial sequence
  F12 RNAi agent antisense strand base sequence
aucgaaaguguugacuccaag

SEQ ID NO: 666 - RNA, 21 nt, Artificial sequence
  F12 RNAi agent antisense strand base sequence
aucgaaaguguugacuccagc

SEQ ID NO: 667 - RNA, 21 nt, Artificial sequence
  F12 RNAi agent antisense strand base sequence
auucaaagcacuauauugagu

SEQ ID NO: 668 - RNA, 21 nt, Artificial sequence
  F12 RNAi agent antisense strand base sequence
auucaaagcacuuuauugagu

SEQ ID NO: 669 - RNA, 21 nt, Artificial sequence
  F12 RNAi agent antisense strand base sequence
auuguacuuaugcuccuuggg

SEQ ID NO: 670 - RNA, 26 nt, Artificial sequence
  F12 RNAi agent antisense strand base sequence
auuuucaaagcacuuuauugaguuca

SEQ ID NO: 671 - RNA, 26 nt, Artificial sequence
  F12 RNAi agent antisense strand base sequence
gcgaugcccaagaaagugaaagacca

SEQ ID NO: 672 - RNA, 21 nt, Artificial sequence
  F12 RNAi agent antisense strand base sequence
uaagcacuuuauugaguuccc

SEQ ID NO: 673 - RNA, 21 nt, Artificial sequence
  F12 RNAi agent antisense strand base sequence
uaagcacuuuauugaguuccu

SEQ ID NO: 674 - RNA, 22 nt, Artificial sequence
  F12 RNAi agent antisense strand base sequence
uaagcacuuuauugaguuccug

SEQ ID NO: 675 - RNA, 22 nt, Artificial sequence
  F12 RNAi agent antisense strand base sequence
uaagcacuuuauugaguuccuu

SEQ ID NO: 676 - RNA, 21 nt, Artificial sequence
  F12 RNAi agent antisense strand base sequence
uaucgaaaguguugacuccaa

SEQ ID NO: 677 - RNA, 22 nt, Artificial sequence
  F12 RNAi agent antisense strand base sequence
uaucgaaaguguugacuccaag

SEQ ID NO: 678 - RNA, 23 nt, Artificial sequence
  F12 RNAi agent antisense strand base sequence
uaucgaaaguguugacuccaagc

SEQ ID NO: 679 - RNA, 21 nt, Artificial sequence
  F12 RNAi agent antisense strand base sequence
uaucgaaaguguugacuccuu

SEQ ID NO: 680 - RNA, 21 nt, Artificial sequence
  F12 RNAi agent antisense strand base sequence
ucaaagcacuuuauugaguuc

SEQ ID NO: 681 - RNA, 22 nt, Artificial sequence
  F12 RNAi agent antisense strand base sequence
ucaaagcacuuuauugaguucu

SEQ ID NO: 682 - RNA, 21 nt, Artificial sequence
  F12 RNAi agent antisense strand base sequence
ucaccuucuugggcuccaaac

SEQ ID NO: 683 - RNA, 23 nt, Artificial sequence
  F12 RNAi agent antisense strand base sequence
ucaccuucuugggcuccaaacac

SEQ ID NO: 684 - RNA, 25 nt, Artificial sequence
  F12 RNAi agent antisense strand base sequence
ucaccuucuugggcuccaaacacgc

SEQ ID NO: 685 - RNA, 21 nt, Artificial sequence
  F12 RNAi agent antisense strand base sequence
ucagcuuuguacuuaugcucc

SEQ ID NO: 686 - RNA, 21 nt, Artificial sequence
  F12 RNAi agent antisense strand base sequence
ucagcuuuguacuuaugcucg

SEQ ID NO: 687 - RNA, 21 nt, Artificial sequence
  F12 RNAi agent antisense strand base sequence
ucagcuuuguacuuaugcucu

SEQ ID NO: 688 - RNA, 21 nt, Artificial sequence
  F12 RNAi agent antisense strand base sequence
ucgaagacagacucuugcguu

SEQ ID NO: 689 - RNA, 19 nt, Artificial sequence
  F12 RNAi agent antisense strand base sequence
ucuuucacuuucuugggcu

SEQ ID NO: 690 - RNA, 20 nt, Artificial sequence
  F12 RNAi agent antisense strand base sequence
ucuuucacuuucuugggcuc

SEQ ID NO: 691 - RNA, 21 nt, Artificial sequence
  F12 RNAi agent antisense strand base sequence
ucuuucacuuucuugggcucc

SEQ ID NO: 692 - RNA, 22 nt, Artificial sequence
  F12 RNAi agent antisense strand base sequence
ucuuucacuuucuugggcucca

SEQ ID NO: 693 - RNA, 23 nt, Artificial sequence
  F12 RNAi agent antisense strand base sequence
ucuuucacuuucuugggcuccaa

SEQ ID NO: 694 - RNA, 24 nt, Artificial sequence
  F12 RNAi agent antisense strand base sequence
ucuuucacuuucuugggcuccaaa

SEQ ID NO: 695 - RNA, 26 nt, Artificial sequence
  F12 RNAi agent antisense strand base sequence
ucuuucacuuucuugggcuccaauca

SEQ ID NO: 696 - RNA, 23 nt, Artificial sequence
  F12 RNAi agent antisense strand base sequence
ucuuucacuuucuugggcuccuu

SEQ ID NO: 697 - RNA, 21 nt, Artificial sequence
  F12 RNAi agent antisense strand base sequence
ucuuucacuuucuugggcuuu

SEQ ID NO: 698 - RNA, 21 nt, Artificial sequence
  F12 RNAi agent antisense strand base sequence
ucuuuguacuuaugcuccucc

SEQ ID NO: 699 - RNA, 21 nt, Artificial sequence
  F12 RNAi agent antisense strand base sequence
ucuuuguacuuaugcuccucg

SEQ ID NO: 700 - RNA, 19 nt, Artificial sequence
  F12 RNAi agent antisense strand base sequence
ugaagcugaggcucaaagc

SEQ ID NO: 701 - RNA, 20 nt, Artificial sequence
  F12 RNAi agent antisense strand base sequence
ugaagcugaggcucaaagca

SEQ ID NO: 702 - RNA, 21 nt, Artificial sequence
  F12 RNAi agent antisense strand base sequence
ugaagcugaggcucaaagcac

SEQ ID NO: 703 - RNA, 22 nt, Artificial sequence
  F12 RNAi agent antisense strand base sequence
ugaagcugaggcucaaagcacu

SEQ ID NO: 704 - RNA, 23 nt, Artificial sequence
  F12 RNAi agent antisense strand base sequence
ugaagcugaggcucaaagcacuu

SEQ ID NO: 705 - RNA, 24 nt, Artificial sequence
  F12 RNAi agent antisense strand base sequence
ugaagcugaggcucaaagcacuuc

SEQ ID NO: 706 - RNA, 26 nt, Artificial sequence
  F12 RNAi agent antisense strand base sequence
ugaagcugaggcucaaagcacuuuca

SEQ ID NO: 707 - RNA, 21 nt, Artificial sequence
  F12 RNAi agent antisense strand base sequence
ugaagcugaggcucaaagcuu

SEQ ID NO: 708 - RNA, 19 nt, Artificial sequence
  F12 RNAi agent antisense strand base sequence
ugagaagcugaggcucaaa

SEQ ID NO: 709 - RNA, 20 nt, Artificial sequence
  F12 RNAi agent antisense strand base sequence
ugagaagcugaggcucaaag

SEQ ID NO: 710 - RNA, 21 nt, Artificial sequence
  F12 RNAi agent antisense strand base sequence
ugagaagcugaggcucaaagc

SEQ ID NO: 711 - RNA, 22 nt, Artificial sequence
  F12 RNAi agent antisense strand base sequence
ugagaagcugaggcucaaagca

SEQ ID NO: 712 - RNA, 23 nt, Artificial sequence
  F12 RNAi agent antisense strand base sequence
ugagaagcugaggcucaaagcac

SEQ ID NO: 713 - RNA, 24 nt, Artificial sequence
  F12 RNAi agent antisense strand base sequence
ugagaagcugaggcucaaagcacu

SEQ ID NO: 714 - RNA, 26 nt, Artificial sequence
  F12 RNAi agent antisense strand base sequence
ugagaagcugaggcucaaagcacuca

SEQ ID NO: 715 - RNA, 23 nt, Artificial sequence
  F12 RNAi agent antisense strand base sequence
ugagaagcugaggcucaaagcuu

SEQ ID NO: 716 - RNA, 21 nt, Artificial sequence
  F12 RNAi agent antisense strand base sequence
ugagaagcugaggcucaaauu

SEQ ID NO: 717 - RNA, 21 nt, Artificial sequence
  F12 RNAi agent antisense strand base sequence
uggaaucgaaaguguugacuc

SEQ ID NO: 718 - RNA, 21 nt, Artificial sequence
  F12 RNAi agent antisense strand base sequence
ugguacauuugugguacagcu

SEQ ID NO: 719 - RNA, 21 nt, Artificial sequence
  F12 RNAi agent antisense strand base sequence
uggucuuucacuuucaugggu

SEQ ID NO: 720 - RNA, 23 nt, Artificial sequence
  F12 RNAi agent antisense strand base sequence
uggucuuucacuuucauggguuu

SEQ ID NO: 721 - RNA, 19 nt, Artificial sequence
  F12 RNAi agent antisense strand base sequence
uggucuuucacuuucuugg

SEQ ID NO: 722 - RNA, 20 nt, Artificial sequence
  F12 RNAi agent antisense strand base sequence
uggucuuucacuuucuuggg

SEQ ID NO: 723 - RNA, 21 nt, Artificial sequence
  F12 RNAi agent antisense strand base sequence
uggucuuucacuuucuuggga

SEQ ID NO: 724 - RNA, 21 nt, Artificial sequence
  F12 RNAi agent antisense strand base sequence
uggucuuucacuuucuugggc

SEQ ID NO: 725 - RNA, 22 nt, Artificial sequence
  F12 RNAi agent antisense strand base sequence
uggucuuucacuuucuugggca

SEQ ID NO: 726 - RNA, 26 nt, Artificial sequence
  F12 RNAi agent antisense strand base sequence
uggucuuucacuuucuugggcaccaa

SEQ ID NO: 727 - RNA, 26 nt, Artificial sequence
  F12 RNAi agent antisense strand base sequence
uggucuuucacuuucuugggcaccac

SEQ ID NO: 728 - RNA, 26 nt, Artificial sequence
  F12 RNAi agent antisense strand base sequence
uggucuuucacuuucuugggcaccgc

SEQ ID NO: 729 - RNA, 26 nt, Artificial sequence
  F12 RNAi agent antisense strand base sequence
uggucuuucacuuucuugggcaccuc

SEQ ID NO: 730 - RNA, 26 nt, Artificial sequence
  F12 RNAi agent antisense strand base sequence
uggucuuucacuuucuugggcaccuu

SEQ ID NO: 731 - RNA, 26 nt, Artificial sequence
  F12 RNAi agent antisense strand base sequence
uggucuuucacuuucuugggcacuau

SEQ ID NO: 732 - RNA, 26 nt, Artificial sequence
  F12 RNAi agent antisense strand base sequence
uggucuuucacuuucuugggcacuca

SEQ ID NO: 733 - RNA, 23 nt, Artificial sequence
  F12 RNAi agent antisense strand base sequence
uggucuuucacuuucuugggcau

SEQ ID NO: 734 - RNA, 24 nt, Artificial sequence
  F12 RNAi agent antisense strand base sequence
uggucuuucacuuucuugggcauc

SEQ ID NO: 735 - RNA, 26 nt, Artificial sequence
  F12 RNAi agent antisense strand base sequence
uggucuuucacuuucuugggcaucgc

SEQ ID NO: 736 - RNA, 26 nt, Artificial sequence
  F12 RNAi agent antisense strand base sequence
uggucuuucacuuucuugggcauuca

SEQ ID NO: 737 - RNA, 24 nt, Artificial sequence
  F12 RNAi agent antisense strand base sequence
uggucuuucacuuucuugggcguu

SEQ ID NO: 738 - RNA, 22 nt, Artificial sequence
  F12 RNAi agent antisense strand base sequence
uggucuuucacuuucuugggcu

SEQ ID NO: 739 - RNA, 23 nt, Artificial sequence
  F12 RNAi agent antisense strand base sequence
uggucuuucacuuucuugggcuc

SEQ ID NO: 740 - RNA, 24 nt, Artificial sequence
  F12 RNAi agent antisense strand base sequence
uggucuuucacuuucuugggcucc

SEQ ID NO: 741 - RNA, 26 nt, Artificial sequence
  F12 RNAi agent antisense strand base sequence
uggucuuucacuuucuugggcuccaa

SEQ ID NO: 742 - RNA, 26 nt, Artificial sequence
  F12 RNAi agent antisense strand base sequence
uggucuuucacuuucuugggcuccgc

SEQ ID NO: 743 - RNA, 25 nt, Artificial sequence
  F12 RNAi agent antisense strand base sequence
uggucuuucacuuucuugggcucgc

SEQ ID NO: 744 - RNA, 26 nt, Artificial sequence
  F12 RNAi agent antisense strand base sequence
uggucuuucacuuucuugggcucuau

SEQ ID NO: 745 - RNA, 26 nt, Artificial sequence
  F12 RNAi agent antisense strand base sequence
uggucuuucacuuucuugggcucuca

SEQ ID NO: 746 - RNA, 23 nt, Artificial sequence
  F12 RNAi agent antisense strand base sequence
uggucuuucacuuucuugggcuu

SEQ ID NO: 747 - RNA, 25 nt, Artificial sequence
  F12 RNAi agent antisense strand base sequence
uggucuuucacuuucuugggcuuau

SEQ ID NO: 748 - RNA, 21 nt, Artificial sequence
  F12 RNAi agent antisense strand base sequence
uggucuuucacuuucuugggu

SEQ ID NO: 749 - RNA, 23 nt, Artificial sequence
  F12 RNAi agent antisense strand base sequence
uggucuuucacuuucuuggguuu

SEQ ID NO: 750 - RNA, 21 nt, Artificial sequence
  F12 RNAi agent antisense strand base sequence
uggucuuucacuuucuugguc

SEQ ID NO: 751 - RNA, 21 nt, Artificial sequence
  F12 RNAi agent antisense strand base sequence
uggucuuucacuuucuugguu

SEQ ID NO: 752 - RNA, 21 nt, Artificial sequence
  F12 RNAi agent antisense strand base sequence
uguacauuugugguacagcug

SEQ ID NO: 753 - RNA, 21 nt, Artificial sequence
  F12 RNAi agent antisense strand base sequence
uguacuuaugcuccuuggggc

SEQ ID NO: 754 - RNA, 19 nt, Artificial sequence
  F12 RNAi agent antisense strand base sequence
ugucuuucacuuucuuggg

SEQ ID NO: 755 - RNA, 20 nt, Artificial sequence
  F12 RNAi agent antisense strand base sequence
ugucuuucacuuucuugggc

SEQ ID NO: 756 - RNA, 21 nt, Artificial sequence
  F12 RNAi agent antisense strand base sequence
ugucuuucacuuucuugggcu

SEQ ID NO: 757 - RNA, 22 nt, Artificial sequence
  F12 RNAi agent antisense strand base sequence
ugucuuucacuuucuugggcuc

SEQ ID NO: 758 - RNA, 23 nt, Artificial sequence
  F12 RNAi agent antisense strand base sequence
ugucuuucacuuucuugggcucc

SEQ ID NO: 759 - RNA, 24 nt, Artificial sequence
  F12 RNAi agent antisense strand base sequence
ugucuuucacuuucuugggcucca

SEQ ID NO: 760 - RNA, 26 nt, Artificial sequence
  F12 RNAi agent antisense strand base sequence
ugucuuucacuuucuugggcuccuca

SEQ ID NO: 761 - RNA, 23 nt, Artificial sequence
  F12 RNAi agent antisense strand base sequence
ugucuuucacuuucuugggcuuu

SEQ ID NO: 762 - RNA, 21 nt, Artificial sequence
  F12 RNAi agent antisense strand base sequence
ugucuuucacuuucuuggguu

SEQ ID NO: 763 - RNA, 21 nt, Artificial sequence
  F12 RNAi agent antisense strand base sequence
uucaaagcacuuuauugagcc

SEQ ID NO: 764 - RNA, 21 nt, Artificial sequence
  F12 RNAi agent antisense strand base sequence
uucaaagcacuuuauugagcu

SEQ ID NO: 765 - RNA, 21 nt, Artificial sequence
  F12 RNAi agent antisense strand base sequence
uucaaagcacuuuauugaguc

SEQ ID NO: 766 - RNA, 22 nt, Artificial sequence
  F12 RNAi agent antisense strand base sequence
uucaaagcacuuuauugagucc

SEQ ID NO: 767 - RNA, 21 nt, Artificial sequence
  F12 RNAi agent antisense strand base sequence
uucaaagcacuuuauugaguu

SEQ ID NO: 768 - RNA, 22 nt, Artificial sequence
  F12 RNAi agent antisense strand base sequence
uucaaagcacuuuauugaguuc

SEQ ID NO: 769 - RNA, 23 nt, Artificial sequence
  F12 RNAi agent antisense strand base sequence
uucaaagcacuuuauugaguucc

SEQ ID NO: 770 - RNA, 23 nt, Artificial sequence
  F12 RNAi agent antisense strand base sequence
uucaaagcacuuuauugaguucc

SEQ ID NO: 771 - RNA, 23 nt, Artificial sequence
  F12 RNAi agent antisense strand base sequence
uucaaagcacuuuauugaguucu

SEQ ID NO: 772 - RNA, 24 nt, Artificial sequence
  F12 RNAi agent antisense strand base sequence
uucaaagcacuuuauugaguucuu

SEQ ID NO: 773 - RNA, 19 nt, Artificial sequence
  F12 RNAi agent antisense strand base sequence
uuggucuuucacuuucuug

SEQ ID NO: 774 - RNA, 20 nt, Artificial sequence
  F12 RNAi agent antisense strand base sequence
uuggucuuucacuuucuugg

SEQ ID NO: 775 - RNA, 21 nt, Artificial sequence
  F12 RNAi agent antisense strand base sequence
uuggucuuucacuuucuuggg

SEQ ID NO: 776 - RNA, 22 nt, Artificial sequence
  F12 RNAi agent antisense strand base sequence
uuggucuuucacuuucuugggc

SEQ ID NO: 777 - RNA, 23 nt, Artificial sequence
  F12 RNAi agent antisense strand base sequence
uuggucuuucacuuucuugggcu

SEQ ID NO: 778 - RNA, 24 nt, Artificial sequence
  F12 RNAi agent antisense strand base sequence
uuggucuuucacuuucuugggcuc

SEQ ID NO: 779 - RNA, 26 nt, Artificial sequence
  F12 RNAi agent antisense strand base sequence
uuggucuuucacuuucuugggcucgc

SEQ ID NO: 780 - RNA, 26 nt, Artificial sequence
  F12 RNAi agent antisense strand base sequence
uuggucuuucacuuucuugggcuuca

SEQ ID NO: 781 - RNA, 23 nt, Artificial sequence
  F12 RNAi agent antisense strand base sequence
uuggucuuucacuuucuuggguu

SEQ ID NO: 782 - RNA, 21 nt, Artificial sequence
  F12 RNAi agent antisense strand base sequence
uuggucuuucacuuucuuguu

SEQ ID NO: 783 - RNA, 21 nt, Artificial sequence
  F12 RNAi agent antisense strand base sequence
uuguacuuaugcuccuugggc

SEQ ID NO: 784 - RNA, 21 nt, Artificial sequence
  F12 RNAi agent antisense strand base sequence
uuguacuuaugcuccuugggg

SEQ ID NO: 785 - RNA, 21 nt, Artificial sequence
  F12 RNAi agent antisense strand base sequence
uuguacuuaugcuccuugggu

SEQ ID NO: 786 - RNA, 22 nt, Artificial sequence
  F12 RNAi agent antisense strand base sequence
uuguacuuaugcuccuuggguu

SEQ ID NO: 787 - RNA, 21 nt, Artificial sequence
  F12 RNAi agent antisense strand base sequence
uuguacuuaugcuccuugguu

SEQ ID NO: 788 - RNA, 21 nt, Artificial sequence
  F12 RNAi agent antisense strand base sequence
uuucaaagcacuauauugagu

SEQ ID NO: 789 - RNA, 23 nt, Artificial sequence
  F12 RNAi agent antisense strand base sequence
uuucaaagcacuauauugaguuc

SEQ ID NO: 790 - RNA, 21 nt, Artificial sequence
  F12 RNAi agent antisense strand base sequence
uuucaaagcacuuuauugagc

SEQ ID NO: 791 - RNA, 22 nt, Artificial sequence
  F12 RNAi agent antisense strand base sequence
uuucaaagcacuuuauugagcc

SEQ ID NO: 792 - RNA, 22 nt, Artificial sequence
  F12 RNAi agent antisense strand base sequence
uuucaaagcacuuuauugagcu

SEQ ID NO: 793 - RNA, 21 nt, Artificial sequence
  F12 RNAi agent antisense strand base sequence
uuucaaagcacuuuauugagu

SEQ ID NO: 794 - RNA, 22 nt, Artificial sequence
  F12 RNAi agent antisense strand base sequence
uuucaaagcacuuuauugaguc

SEQ ID NO: 795 - RNA, 23 nt, Artificial sequence
  F12 RNAi agent antisense strand base sequence
uuucaaagcacuuuauugagucc

SEQ ID NO: 796 - RNA, 22 nt, Artificial sequence
  F12 RNAi agent antisense strand base sequence
uuucaaagcacuuuauugaguu

SEQ ID NO: 797 - RNA, 23 nt, Artificial sequence
  F12 RNAi agent antisense strand base sequence
uuucaaagcacuuuauugaguuc

SEQ ID NO: 798 - RNA, 21 nt, Artificial sequence
  F12 RNAi agent antisense strand base sequence
uuucaaagcacuuuauugauu

SEQ ID NO: 799 - RNA, 21 nt, Artificial sequence
  F12 RNAi agent antisense strand base sequence
uuucacuuucuugggcuccaa

SEQ ID NO: 800 - RNA, 23 nt, Artificial sequence
  F12 RNAi agent antisense strand base sequence
uuucacuuucuugggcuccaaac

SEQ ID NO: 801 - RNA, 21 nt, Artificial sequence
  F12 RNAi agent antisense strand base sequence
uuucacuuucuugggcuccuu

SEQ ID NO: 802 - RNA, 19 nt, Artificial sequence
  F12 RNAi agent antisense strand base sequence
uuuguacuuaugcuccuug

SEQ ID NO: 803 - RNA, 20 nt, Artificial sequence
  F12 RNAi agent antisense strand base sequence
uuuguacuuaugcuccuugg

SEQ ID NO: 804 - RNA, 21 nt, Artificial sequence
  F12 RNAi agent antisense strand base sequence
uuuguacuuaugcuccuuggc

SEQ ID NO: 805 - RNA, 21 nt, Artificial sequence
  F12 RNAi agent antisense strand base sequence
uuuguacuuaugcuccuuggg

SEQ ID NO: 806 - RNA, 22 nt, Artificial sequence
  F12 RNAi agent antisense strand base sequence
uuuguacuuaugcuccuugggg

SEQ ID NO: 807 - RNA, 23 nt, Artificial sequence
  F12 RNAi agent antisense strand base sequence
uuuguacuuaugcuccuuggggu

SEQ ID NO: 808 - RNA, 23 nt, Artificial sequence
  F12 RNAi agent antisense strand base sequence
uuuguacuuaugcuccuuggguu

SEQ ID NO: 809 - RNA, 21 nt, Artificial sequence
  F12 RNAi agent antisense strand base sequence
uuuguacuuaugcuccuuggu

SEQ ID NO: 810 - RNA, 20 nt, Artificial sequence
  F12 RNAi agent antisense strand base sequence
uuuguacuuaugcuccuugu

SEQ ID NO: 811 - RNA, 21 nt, Artificial sequence
  F12 RNAi agent antisense strand base sequence
uuuguacuuaugcuccuuguu

SEQ ID NO: 812 - RNA, 21 nt, Artificial sequence
  F12 RNAi agent antisense strand base sequence
uuuuguacuuaugcuccuugc

SEQ ID NO: 813 - RNA, 21 nt, Artificial sequence
  F12 RNAi agent antisense strand base sequence
uuuuucaaagcacuuuaucga

SEQ ID NO: 814 - RNA, 19 nt, Artificial sequence
  F12 RNAi agent antisense strand base sequence
uuuuucaaagcacuuuauu

SEQ ID NO: 815 - RNA, 20 nt, Artificial sequence
  F12 RNAi agent antisense strand base sequence
uuuuucaaagcacuuuauug

SEQ ID NO: 816 - RNA, 21 nt, Artificial sequence
  F12 RNAi agent antisense strand base sequence
uuuuucaaagcacuuuauuga

SEQ ID NO: 817 - RNA, 22 nt, Artificial sequence
  F12 RNAi agent antisense strand base sequence
uuuuucaaagcacuuuauugag

SEQ ID NO: 818 - RNA, 23 nt, Artificial sequence
  F12 RNAi agent antisense strand base sequence
uuuuucaaagcacuuuauugagu

SEQ ID NO: 819 - RNA, 24 nt, Artificial sequence
  F12 RNAi agent antisense strand base sequence
uuuuucaaagcacuuuauugaguu

SEQ ID NO: 820 - RNA, 26 nt, Artificial sequence
  F12 RNAi agent antisense strand base sequence
uuuuucaaagcacuuuauugaguuau

SEQ ID NO: 821 - RNA, 26 nt, Artificial sequence
  F12 RNAi agent antisense strand base sequence
uuuuucaaagcacuuuauugaguuca

SEQ ID NO: 822 - RNA, 23 nt, Artificial sequence
  F12 RNAi agent antisense strand base sequence
uuuuucaaagcacuuuauugauu

SEQ ID NO: 823 - RNA, 21 nt, Artificial sequence
  F12 RNAi agent antisense strand base sequence
uuuuucaaagcacuuuauugc

SEQ ID NO: 824 - RNA, 21 nt, Artificial sequence
  F12 RNAi agent antisense strand base sequence
uuuuucaaagcacuuuauugu

SEQ ID NO: 825 - RNA, 21 nt, Artificial sequence
  F12 RNAi agent antisense strand base sequence
uuuuucaaagcacuuuauuuu

SEQ ID NO: 826 - RNA, 25 nt, Artificial sequence
  F12 RNAi agent sense strand base sequence
aaagcccaagaaagugaaagacauu

SEQ ID NO: 827 - RNA, 21 nt, Artificial sequence
  F12 RNAi agent sense strand base sequence
aaccaagaaagugaaagacca

SEQ ID NO: 828 - RNA, 25 nt, Artificial sequence
  F12 RNAi agent sense strand base sequence
aacccaagaaagugaaagaccaauu

SEQ ID NO: 829 - RNA, 21 nt, Artificial sequence
  F12 RNAi agent sense strand base sequence
aacucaauaaagugcuuugaa

SEQ ID NO: 830 - RNA, 22 nt, Artificial sequence
  F12 RNAi agent sense strand base sequence
aacucaauaaagugcuuugaaa

SEQ ID NO: 831 - RNA, 23 nt, Artificial sequence
  F12 RNAi agent sense strand base sequence
aacucaauaaagugcuuugaauu

SEQ ID NO: 832 - RNA, 23 nt, Artificial sequence
  F12 RNAi agent sense strand base sequence
aagcccaagaaagugaaagacca

SEQ ID NO: 833 - RNA, 25 nt, Artificial sequence
  F12 RNAi agent sense strand base sequence
aagcccaagaaagugaaagaccauu

SEQ ID NO: 834 - RNA, 21 nt, Artificial sequence
  F12 RNAi agent sense strand base sequence
aagcuuugagccucagcuuca

SEQ ID NO: 835 - RNA, 25 nt, Artificial sequence
  F12 RNAi agent sense strand base sequence
aagcuuugagccucagcuucucauu

SEQ ID NO: 836 - RNA, 25 nt, Artificial sequence
  F12 RNAi agent sense strand base sequence
aaggagcccaagaaagugaaagauu

SEQ ID NO: 837 - RNA, 26 nt, Artificial sequence
  F12 RNAi agent sense strand base sequence
aaggugcccaagaaagugaaagacca

SEQ ID NO: 838 - RNA, 25 nt, Artificial sequence
  F12 RNAi agent sense strand base sequence
aagugcuuugagccucagcuucauu

SEQ ID NO: 839 - RNA, 21 nt, Artificial sequence
  F12 RNAi agent sense strand base sequence
aauaaagugcuuugaaaaauu

SEQ ID NO: 840 - RNA, 25 nt, Artificial sequence
  F12 RNAi agent sense strand base sequence
aaucaauaaagugcuuugaaaaauu

SEQ ID NO: 841 - RNA, 21 nt, Artificial sequence
  F12 RNAi agent sense strand base sequence
acaauaaagugcuuugaaaaa

SEQ ID NO: 842 - RNA, 23 nt, Artificial sequence
  F12 RNAi agent sense strand base sequence
acaauaaagugcuuugaaaaauu

SEQ ID NO: 843 - RNA, 21 nt, Artificial sequence
  F12 RNAi agent sense strand base sequence
acacaagaaagugaaagacca

SEQ ID NO: 844 - RNA, 21 nt, Artificial sequence
  F12 RNAi agent sense strand base sequence
accaaggagcauaaguacaaa

SEQ ID NO: 845 - RNA, 21 nt, Artificial sequence
  F12 RNAi agent sense strand base sequence
acccaaggagcauaaguacaa

SEQ ID NO: 846 - RNA, 21 nt, Artificial sequence
  F12 RNAi agent sense strand base sequence
acucaauaaagugcuuugaaa

SEQ ID NO: 847 - RNA, 21 nt, Artificial sequence
  F12 RNAi agent sense strand base sequence
acucaauaaagugcuuugaau

SEQ ID NO: 848 - RNA, 22 nt, Artificial sequence
  F12 RNAi agent sense strand base sequence
agaacucaauaaagugcuuuga

SEQ ID NO: 849 - RNA, 23 nt, Artificial sequence
  F12 RNAi agent sense strand base sequence
agaacucaauaaagugcuuugaa

SEQ ID NO: 850 - RNA, 21 nt, Artificial sequence
  F12 RNAi agent sense strand base sequence
agagcauaaguacaaagcuga

SEQ ID NO: 851 - RNA, 21 nt, Artificial sequence
  F12 RNAi agent sense strand base sequence
agcccaagaaagugaaagauu

SEQ ID NO: 852 - RNA, 21 nt, Artificial sequence
  F12 RNAi agent sense strand base sequence
agcucaauaaagugcuuugaa

SEQ ID NO: 853 - RNA, 22 nt, Artificial sequence
  F12 RNAi agent sense strand base sequence
agcucaauaaagugcuuugaaa

SEQ ID NO: 854 - RNA, 21 nt, Artificial sequence
  F12 RNAi agent sense strand base sequence
agcuguaccacaaauguacca

SEQ ID NO: 855 - RNA, 21 nt, Artificial sequence
  F12 RNAi agent sense strand base sequence
aggaacucaauaaagugcuua

SEQ ID NO: 856 - RNA, 23 nt, Artificial sequence
  F12 RNAi agent sense strand base sequence
aggaacucaauaaagugcuuauu

SEQ ID NO: 857 - RNA, 21 nt, Artificial sequence
  F12 RNAi agent sense strand base sequence
aggaacucaauaaagugcuuu

SEQ ID NO: 858 - RNA, 22 nt, Artificial sequence
  F12 RNAi agent sense strand base sequence
aucaauaaagugcuuugaaaaa

SEQ ID NO: 859 - RNA, 21 nt, Artificial sequence
  F12 RNAi agent sense strand base sequence
caagaaagugaaagaccaauu

SEQ ID NO: 860 - RNA, 19 nt, Artificial sequence
  F12 RNAi agent sense strand base sequence
caaggagcauaaguacaaa

SEQ ID NO: 861 - RNA, 21 nt, Artificial sequence
  F12 RNAi agent sense strand base sequence
caaggagcauaaguacaaauu

SEQ ID NO: 862 - RNA, 21 nt, Artificial sequence
  F12 RNAi agent sense strand base sequence
cagcuguaccacaaauguaca

SEQ ID NO: 863 - RNA, 22 nt, Artificial sequence
  F12 RNAi agent sense strand base sequence
caggaacucaauaaagugcuua

SEQ ID NO: 864 - RNA, 21 nt, Artificial sequence
  F12 RNAi agent sense strand base sequence
ccaagaaagugaaagaccauu

SEQ ID NO: 865 - RNA, 20 nt, Artificial sequence
  F12 RNAi agent sense strand base sequence
ccaaggagcauaaguacaaa

SEQ ID NO: 866 - RNA, 21 nt, Artificial sequence
  F12 RNAi agent sense strand base sequence
ccaaggagcauaaguacaauu

SEQ ID NO: 867 - RNA, 21 nt, Artificial sequence
  F12 RNAi agent sense strand base sequence
cccaagaaagugaaagacauu

SEQ ID NO: 868 - RNA, 21 nt, Artificial sequence
  F12 RNAi agent sense strand base sequence
cccaaggagcauaaguacaaa

SEQ ID NO: 869 - RNA, 23 nt, Artificial sequence
  F12 RNAi agent sense strand base sequence
cccaaggagcauaaguacaaauu

SEQ ID NO: 870 - RNA, 21 nt, Artificial sequence
  F12 RNAi agent sense strand base sequence
cccaaggagcauaaguacaau

SEQ ID NO: 871 - RNA, 22 nt, Artificial sequence
  F12 RNAi agent sense strand base sequence
cccaaggagcauaaguacaauu

SEQ ID NO: 872 - RNA, 21 nt, Artificial sequence
  F12 RNAi agent sense strand base sequence
ccccaaggagcauaaguacaa

SEQ ID NO: 873 - RNA, 22 nt, Artificial sequence
  F12 RNAi agent sense strand base sequence
ccccaaggagcauaaguacaaa

SEQ ID NO: 874 - RNA, 21 nt, Artificial sequence
  F12 RNAi agent sense strand base sequence
cgagcauaaguacaaagcuga

SEQ ID NO: 875 - RNA, 21 nt, Artificial sequence
  F12 RNAi agent sense strand base sequence
cgaggagcauaaguacaaaga

SEQ ID NO: 876 - RNA, 21 nt, Artificial sequence
  F12 RNAi agent sense strand base sequence
cgcaagagucugucuucgauu

SEQ ID NO: 877 - RNA, 19 nt, Artificial sequence
  F12 RNAi agent sense strand base sequence
cucaauaaagugcuuugaa

SEQ ID NO: 878 - RNA, 22 nt, Artificial sequence
  F12 RNAi agent sense strand base sequence
cucaauaaagugcuuugaaaaa

SEQ ID NO: 879 - RNA, 21 nt, Artificial sequence
  F12 RNAi agent sense strand base sequence
cucaauaaagugcuuugaauu

SEQ ID NO: 880 - RNA, 21 nt, Artificial sequence
  F12 RNAi agent sense strand base sequence
cuuggagucaacacuuucgau

SEQ ID NO: 881 - RNA, 22 nt, Artificial sequence
  F12 RNAi agent sense strand base sequence
cuuggagucaacacuuucgaua

SEQ ID NO: 882 - RNA, 22 nt, Artificial sequence
  F12 RNAi agent sense strand base sequence
gaacucaauaaagugcugugaa

SEQ ID NO: 883 - RNA, 21 nt, Artificial sequence
  F12 RNAi agent sense strand base sequence
gaacucaauaaagugcuuauu

SEQ ID NO: 884 - RNA, 21 nt, Artificial sequence
  F12 RNAi agent sense strand base sequence
gaacucaauaaagugcuuuga

SEQ ID NO: 885 - RNA, 22 nt, Artificial sequence
  F12 RNAi agent sense strand base sequence
gaacucaauaaagugcuuugaa

SEQ ID NO: 886 - RNA, 23 nt, Artificial sequence
  F12 RNAi agent sense strand base sequence
gaacucaauaaagugcuuugaaa

SEQ ID NO: 887 - RNA, 24 nt, Artificial sequence
  F12 RNAi agent sense strand base sequence
gaacucaauaaagugcuuugaauu

SEQ ID NO: 888 - RNA, 21 nt, Artificial sequence
  F12 RNAi agent sense strand base sequence
gaccaagaaagugaaagacca

SEQ ID NO: 889 - RNA, 21 nt, Artificial sequence
  F12 RNAi agent sense strand base sequence
gacucaauaaagugcuuugaa

SEQ ID NO: 890 - RNA, 22 nt, Artificial sequence
  F12 RNAi agent sense strand base sequence
gacucaauaaagugcuuugaaa

SEQ ID NO: 891 - RNA, 23 nt, Artificial sequence
  F12 RNAi agent sense strand base sequence
gagcccaagaaagugaaagacca

SEQ ID NO: 892 - RNA, 26 nt, Artificial sequence
  F12 RNAi agent sense strand base sequence
gaggugcccaagaaagugaaagacca

SEQ ID NO: 893 - RNA, 21 nt, Artificial sequence
  F12 RNAi agent sense strand base sequence
gagucaacacuuucgauucca

SEQ ID NO: 894 - RNA, 21 nt, Artificial sequence
  F12 RNAi agent sense strand base sequence
gcaaggagcauaaguacaaaa

SEQ ID NO: 895 - RNA, 21 nt, Artificial sequence
  F12 RNAi agent sense strand base sequence
gcaauaaagugcuuugaaaaa

SEQ ID NO: 896 - RNA, 21 nt, Artificial sequence
  F12 RNAi agent sense strand base sequence
gccaaggagcauaaguacaaa

SEQ ID NO: 897 - RNA, 21 nt, Artificial sequence
  F12 RNAi agent sense strand base sequence
  modified_base 15: n = i (inosine)
gccaaggagcauaanuacaaa

SEQ ID NO: 898 - RNA, 21 nt, Artificial sequence
  F12 RNAi agent sense strand base sequence
gcccaagaaagugaaagacca

SEQ ID NO: 899 - RNA, 21 nt, Artificial sequence
  F12 RNAi agent sense strand base sequence
gcccaaggagcauaaguacaa

SEQ ID NO: 900 - RNA, 21 nt, Artificial sequence
  F12 RNAi agent sense strand base sequence
gccccaaggagcauaaguaca

SEQ ID NO: 901 - RNA, 25 nt, Artificial sequence
  F12 RNAi agent sense strand base sequence
gcgagcccaagaaagugaaagacca

SEQ ID NO: 902 - RNA, 26 nt, Artificial sequence
  F12 RNAi agent sense strand base sequence
gcgagcccaagaaagugaaagaccaa

SEQ ID NO: 903 - RNA, 27 nt, Artificial sequence
  F12 RNAi agent sense strand base sequence
gcgagcccaagaaagugaaagaccaaa

SEQ ID NO: 904 - RNA, 25 nt, Artificial sequence
  F12 RNAi agent sense strand base sequence
gcgaugcccaagaaagugaaagacc

SEQ ID NO: 905 - RNA, 26 nt, Artificial sequence
  F12 RNAi agent sense strand base sequence
gcgaugcccaagaaagugaaagacca

SEQ ID NO: 906 - DNA, 26 bp, Artificial sequence
  F12 RNAi agent sense strand base sequence
gcgaugcccaagaaagugaaagacct

SEQ ID NO: 907 - RNA, 26 nt, Artificial sequence
  F12 RNAi agent sense strand base sequence
gcggagcccaagaaagugaaagacca

SEQ ID NO: 908 - RNA, 25 nt, Artificial sequence
  F12 RNAi agent sense strand base sequence
gcguguuuggagcccaagaaaguga

SEQ ID NO: 909 - RNA, 26 nt, Artificial sequence
  F12 RNAi agent sense strand base sequence
gcguguuuggagcccaagaaagugaa

SEQ ID NO: 910 - RNA, 21 nt, Artificial sequence
  F12 RNAi agent sense strand base sequence
gcucaauaaagugcuuugaaa

SEQ ID NO: 911 - RNA, 21 nt, Artificial sequence
  F12 RNAi agent sense strand base sequence
gcuggagucaacacuuucgau

SEQ ID NO: 912 - RNA, 23 nt, Artificial sequence
  F12 RNAi agent sense strand base sequence
gcuuggagucaacacuuucgaua

SEQ ID NO: 913 - RNA, 19 nt, Artificial sequence
  F12 RNAi agent sense strand base sequence
gcuuugagccucagcuuca

SEQ ID NO: 914 - RNA, 21 nt, Artificial sequence
  F12 RNAi agent sense strand base sequence
gcuuugagccucagcuucauu

SEQ ID NO: 915 - RNA, 20 nt, Artificial sequence
  F12 RNAi agent sense strand base sequence
ggaacucaauaaagugcuua

SEQ ID NO: 916 - RNA, 22 nt, Artificial sequence
  F12 RNAi agent sense strand base sequence
ggaacucaauaaagugcuuuga

SEQ ID NO: 917 - RNA, 23 nt, Artificial sequence
  F12 RNAi agent sense strand base sequence
ggaacucaauaaagugcuuugaa

SEQ ID NO: 918 - RNA, 22 nt, Artificial sequence
  F12 RNAi agent sense strand base sequence
ggacucaauaaagugcuuugaa

SEQ ID NO: 919 - RNA, 23 nt, Artificial sequence
  F12 RNAi agent sense strand base sequence
ggacucaauaaagugcuuugaaa

SEQ ID NO: 920 - RNA, 21 nt, Artificial sequence
  F12 RNAi agent sense strand base sequence
ggagcauaaguacaaagcuga

SEQ ID NO: 921 - RNA, 19 nt, Artificial sequence
  F12 RNAi agent sense strand base sequence
ggagcccaagaaagugaaa

SEQ ID NO: 922 - RNA, 21 nt, Artificial sequence
  F12 RNAi agent sense strand base sequence
ggagcccaagaaagugaaauu

SEQ ID NO: 923 - RNA, 21 nt, Artificial sequence
  F12 RNAi agent sense strand base sequence
ggaggagcauaaguacaaaga

SEQ ID NO: 924 - RNA, 19 nt, Artificial sequence
  F12 RNAi agent sense strand base sequence
ggagucaacacuuucgaua

SEQ ID NO: 925 - RNA, 21 nt, Artificial sequence
  F12 RNAi agent sense strand base sequence
ggagucaacacuuucgauauu

SEQ ID NO: 926 - RNA, 21 nt, Artificial sequence
  F12 RNAi agent sense strand base sequence
ggcucaauaaagugcuuugaa

SEQ ID NO: 927 - RNA, 22 nt, Artificial sequence
  F12 RNAi agent sense strand base sequence
ggcucaauaaagugcuuugaaa

SEQ ID NO: 928 - RNA, 21 nt, Artificial sequence
  F12 RNAi agent sense strand base sequence
gggaacucaauaaagugcuua

SEQ ID NO: 929 - RNA, 21 nt, Artificial sequence
  F12 RNAi agent sense strand base sequence
gugcuuugagccucagcuuca

SEQ ID NO: 930 - RNA, 21 nt, Artificial sequence
  F12 RNAi agent sense strand base sequence
guggagucaacacuuucgauu

SEQ ID NO: 931 - RNA, 26 nt, Artificial sequence
  F12 RNAi agent sense strand base sequence
guggugcccaagaaagugaaagacca

SEQ ID NO: 932 - RNA, 26 nt, Artificial sequence
  F12 RNAi agent sense strand base sequence
uauaugcccaagaaagugaaagacca

SEQ ID NO: 933 - RNA, 26 nt, Artificial sequence
  F12 RNAi agent sense strand base sequence
uauaugcccaagaaagugaaagacca

SEQ ID NO: 934 - RNA, 19 nt, Artificial sequence
  F12 RNAi agent sense strand base sequence
ucaauaaagugcuuugaaa

SEQ ID NO: 935 - RNA, 21 nt, Artificial sequence
  F12 RNAi agent sense strand base sequence
ucaauaaagugcuuugaaaaa

SEQ ID NO: 936 - RNA, 21 nt, Artificial sequence
  F12 RNAi agent sense strand base sequence
ucaauaaagugcuuugaaauu

SEQ ID NO: 937 - RNA, 21 nt, Artificial sequence
  F12 RNAi agent sense strand base sequence
ucgauaaagugcuuugaaaaa

SEQ ID NO: 938 - RNA, 26 nt, Artificial sequence
  F12 RNAi agent sense strand base sequence
ugaaagugcuuugagccucagcuuca

SEQ ID NO: 939 - RNA, 26 nt, Artificial sequence
  F12 RNAi agent sense strand base sequence
ugaacucaauaaagugcuuugaaaaa

SEQ ID NO: 940 - RNA, 28 nt, Artificial sequence
  F12 RNAi agent sense strand base sequence
ugaacucaauaaagugcuuugaaaaauu

SEQ ID NO: 941 - DNA, 26 bp, Artificial sequence
  F12 RNAi agent sense strand base sequence
ugaacucaauaaagugcuuugaaaat

SEQ ID NO: 942 - RNA, 26 nt, Artificial sequence
  F12 RNAi agent sense strand base sequence
ugaagcccaagaaagugaaagaccaa

SEQ ID NO: 943 - RNA, 26 nt, Artificial sequence
  F12 RNAi agent sense strand base sequence
ugaaugcccaagaaagugaaagacca

SEQ ID NO: 944 - RNA, 26 nt, Artificial sequence
  F12 RNAi agent sense strand base sequence
ugaggagcccaagaaagugaaagaca

SEQ ID NO: 945 - RNA, 26 nt, Artificial sequence
  F12 RNAi agent sense strand base sequence
ugagugcccaagaaagugaaagacca

SEQ ID NO: 946 - RNA, 26 nt, Artificial sequence
  F12 RNAi agent sense strand base sequence
ugagugcuuugagccucagcuucuca

SEQ ID NO: 947 - RNA, 26 nt, Artificial sequence
  F12 RNAi agent sense strand base sequence
ugauuggagcccaagaaagugaaaga

SEQ ID NO: 948 - RNA, 21 nt, Artificial sequence
  F12 RNAi agent sense strand base sequence
uuggagcccaagaaagugaaa

SEQ ID NO: 949 - RNA, 21 nt, Artificial sequence
  F12 RNAi agent sense strand base sequence
uuggagucaacacuuucgaua

SEQ ID NO: 950 - RNA, 26 nt, Artificial sequence
  F12 RNAi agent sense strand base sequence
uuggugcccaagaaagugaaagacca

SEQ ID NO: 951 - RNA, 21 nt, Artificial sequence
  F12 RNAi agent sense strand base sequence
uuugagccucagcuucucauu

SEQ ID NO: 952 - RNA, 21 nt, Artificial sequence
  F12 RNAi agent antisense strand modified sequence
uaucgaaaguguugacuccuu

SEQ ID NO: 953 - RNA, 21 nt, Artificial sequence
  F12 RNAi agent antisense strand modified sequence
uaucgaaaguguugacuccuu

SEQ ID NO: 954 - RNA, 21 nt, Artificial sequence
  F12 RNAi agent antisense strand modified sequence
uaucgaaaguguugacuccuu

SEQ ID NO: 955 - RNA, 21 nt, Artificial sequence
  F12 RNAi agent antisense strand modified sequence
uaucgaaaguguugacuccuu

SEQ ID NO: 956 - RNA, 21 nt, Artificial sequence
  F12 RNAi agent antisense strand modified sequence
uaucgaaaguguugacuccaa

SEQ ID NO: 957 - RNA, 21 nt, Artificial sequence
  F12 RNAi agent antisense strand modified sequence
uaucgaaaguguugacuccuu

SEQ ID NO: 958 - RNA, 21 nt, Artificial sequence
  F12 RNAi agent antisense strand modified sequence
uaucgaaaguguugacuccaa

SEQ ID NO: 959 - RNA, 23 nt, Artificial sequence
  F12 RNAi agent antisense strand modified sequence
uaucgaaaguguugacuccaacg

SEQ ID NO: 960 - RNA, 21 nt, Artificial sequence
  F12 RNAi agent antisense strand modified sequence
uguacuuaugcuccuuggguu

SEQ ID NO: 961 - RNA, 21 nt, Artificial sequence
  F12 RNAi agent antisense strand modified sequence
uguacuuaugcuccuuggguu

SEQ ID NO: 962 - RNA, 21 nt, Artificial sequence
  F12 RNAi agent antisense strand modified sequence
uguacuuaugcuccuuggguu

SEQ ID NO: 963 - RNA, 21 nt, Artificial sequence
  F12 RNAi agent antisense strand modified sequence
uguacuuaugcuccuuggguu

SEQ ID NO: 964 - RNA, 21 nt, Artificial sequence
  F12 RNAi agent antisense strand modified sequence
uuguacuuaugcuccuugguu

SEQ ID NO: 965 - RNA, 21 nt, Artificial sequence
  F12 RNAi agent antisense strand modified sequence
uuguacuuaugcuccuugguu

SEQ ID NO: 966 - RNA, 21 nt, Artificial sequence
  F12 RNAi agent antisense strand modified sequence
uuguacuuaugcuccuugguu

SEQ ID NO: 967 - RNA, 21 nt, Artificial sequence
  F12 RNAi agent antisense strand modified sequence
uuguacuuaugcuccuugguu

SEQ ID NO: 968 - RNA, 21 nt, Artificial sequence
  F12 RNAi agent antisense strand modified sequence
uuguacuuaugcuccuugggu

SEQ ID NO: 969 - RNA, 21 nt, Artificial sequence
  F12 RNAi agent antisense strand modified sequence
uuguacuuaugcuccuugggg

SEQ ID NO: 970 - RNA, 21 nt, Artificial sequence
  F12 RNAi agent antisense strand modified sequence
uuuguacuuaugcuccuuguu

SEQ ID NO: 971 - RNA, 21 nt, Artificial sequence
  F12 RNAi agent antisense strand modified sequence
uuuguacuuaugcuccuuguu

SEQ ID NO: 972 - RNA, 21 nt, Artificial sequence
  F12 RNAi agent antisense strand modified sequence
uuuguacuuaugcuccuuguu

SEQ ID NO: 973 - RNA, 21 nt, Artificial sequence
  F12 RNAi agent antisense strand modified sequence
uuuguacuuaugcuccuugcc

SEQ ID NO: 974 - RNA, 21 nt, Artificial sequence
  F12 RNAi agent antisense strand modified sequence
uuuguacuuaugcuccuugcc

SEQ ID NO: 975 - RNA, 21 nt, Artificial sequence
  F12 RNAi agent antisense strand modified sequence
ucagcuuuguacuuaugcuuu

SEQ ID NO: 976 - RNA, 21 nt, Artificial sequence
  F12 RNAi agent antisense strand modified sequence
ucagcuuuguacuuaugcucc

SEQ ID NO: 977 - RNA, 21 nt, Artificial sequence
  F12 RNAi agent antisense strand modified sequence
uuuguggguacauuugugguu

SEQ ID NO: 978 - RNA, 21 nt, Artificial sequence
  F12 RNAi agent antisense strand modified sequence
uugucguuguccggguuccuu

SEQ ID NO: 979 - RNA, 21 nt, Artificial sequence
  F12 RNAi agent antisense strand modified sequence
augucguuguccggguuccuu

SEQ ID NO: 980 - RNA, 21 nt, Artificial sequence
  F12 RNAi agent antisense strand modified sequence
ucgaagacagacucuugcguu

SEQ ID NO: 981 - RNA, 21 nt, Artificial sequence
  F12 RNAi agent antisense strand modified sequence
ucgaagacagacucuugcguu

SEQ ID NO: 982 - RNA, 21 nt, Artificial sequence
  F12 RNAi agent antisense strand modified sequence
ucgaagacagacucuugcguu

SEQ ID NO: 983 - RNA, 21 nt, Artificial sequence
  F12 RNAi agent antisense strand modified sequence
ucgaagacagacucuugcguu

SEQ ID NO: 984 - RNA, 21 nt, Artificial sequence
  F12 RNAi agent antisense strand modified sequence
acguaaggcgacaggagcguu

SEQ ID NO: 985 - RNA, 21 nt, Artificial sequence
  F12 RNAi agent antisense strand modified sequence
ucguaaggcgacaggagcguu

SEQ ID NO: 986 - RNA, 21 nt, Artificial sequence
  F12 RNAi agent antisense strand modified sequence
ucguaaggcgacaggagcguu

SEQ ID NO: 987 - RNA, 21 nt, Artificial sequence
  F12 RNAi agent antisense strand modified sequence
ucguaaggcgacaggagcguu

SEQ ID NO: 988 - RNA, 21 nt, Artificial sequence
  F12 RNAi agent antisense strand modified sequence
ucguaaggcgacaggagcguu

SEQ ID NO: 989 - RNA, 21 nt, Artificial sequence
  F12 RNAi agent sense strand modified sequence
ggagucaacacuuucgauauu

SEQ ID NO: 990 - RNA, 21 nt, Artificial sequence
  F12 RNAi agent sense strand modified sequence
ggagucaacacuuucgauauu

SEQ ID NO: 991 - RNA, 21 nt, Artificial sequence
  F12 RNAi agent sense strand modified sequence
ggagucaacacuuucgauauu

SEQ ID NO: 992 - RNA, 21 nt, Artificial sequence
  F12 RNAi agent sense strand modified sequence
ggagucaacacuuucgauauu

SEQ ID NO: 993 - RNA, 21 nt, Artificial sequence
  F12 RNAi agent sense strand modified sequence
ggagucaacacuuucgauauu

SEQ ID NO: 994 - RNA, 21 nt, Artificial sequence
  F12 RNAi agent sense strand modified sequence
ggagucaacacuuucgauauu

SEQ ID NO: 995 - RNA, 21 nt, Artificial sequence
  F12 RNAi agent sense strand modified sequence
ggagucaacacuuucgauauu

SEQ ID NO: 996 - RNA, 21 nt, Artificial sequence
  F12 RNAi agent sense strand modified sequence
uuggagucaacacuuucgaua

SEQ ID NO: 997 - RNA, 21 nt, Artificial sequence
  F12 RNAi agent sense strand modified sequence
uuggagucaacacuuucgaua

SEQ ID NO: 998 - RNA, 21 nt, Artificial sequence
  F12 RNAi agent sense strand modified sequence
cccaaggagcauaaguacauu

SEQ ID NO: 999 - RNA, 21 nt, Artificial sequence
  F12 RNAi agent sense strand modified sequence
cccaaggagcauaaguacauu

SEQ ID NO: 1000 - RNA, 21 nt, Artificial sequence
  F12 RNAi agent sense strand modified sequence
cccaaggagcauaaguacauu

SEQ ID NO: 1001 - RNA, 21 nt, Artificial sequence
  F12 RNAi agent sense strand modified sequence
cccaaggagcauaaguacauu

SEQ ID NO: 1002 - RNA, 21 nt, Artificial sequence
  F12 RNAi agent sense strand modified sequence
ccaaggagcauaaguacaauu

SEQ ID NO: 1003 - RNA, 21 nt, Artificial sequence
  F12 RNAi agent sense strand modified sequence
ccaaggagcauaaguacaauu

SEQ ID NO: 1004 - RNA, 21 nt, Artificial sequence
  F12 RNAi agent sense strand modified sequence
ccaaggagcauaaguacaauu

SEQ ID NO: 1005 - RNA, 21 nt, Artificial sequence
  F12 RNAi agent sense strand modified sequence
ccaaggagcauaaguacaauu

SEQ ID NO: 1006 - RNA, 21 nt, Artificial sequence
  F12 RNAi agent sense strand modified sequence
acccaaggagcauaaguacaa

SEQ ID NO: 1007 - RNA, 21 nt, Artificial sequence
  F12 RNAi agent sense strand modified sequence
ccccaaggagcauaaguacaa

SEQ ID NO: 1008 - RNA, 21 nt, Artificial sequence
  F12 RNAi agent sense strand modified sequence
caaggagcauaaguacaaauu

SEQ ID NO: 1009 - RNA, 21 nt, Artificial sequence
  F12 RNAi agent sense strand modified sequence
caaggagcauaaguacaaauu

SEQ ID NO: 1010 - RNA, 21 nt, Artificial sequence
  F12 RNAi agent sense strand modified sequence
caaggagcauaaguacaaauu

SEQ ID NO: 1011 - RNA, 21 nt, Artificial sequence
  F12 RNAi agent sense strand modified sequence
ggcaaggagcauaaguacaaa

SEQ ID NO: 1012 - RNA, 21 nt, Artificial sequence
  F12 RNAi agent sense strand modified sequence
ggcaaggagcauaaguacaaa

SEQ ID NO: 1013 - RNA, 21 nt, Artificial sequence
  F12 RNAi agent sense strand modified sequence
agcauaaguacaaagcugauu

SEQ ID NO: 1014 - RNA, 21 nt, Artificial sequence
  F12 RNAi agent sense strand modified sequence
ggagcauaaguacaaagcuga

SEQ ID NO: 1015 - RNA, 21 nt, Artificial sequence
  F12 RNAi agent sense strand modified sequence
ccacaaauguacccacaaauu

SEQ ID NO: 1016 - RNA, 21 nt, Artificial sequence
  F12 RNAi agent sense strand modified sequence
ggaacccggacaacgacaauu

SEQ ID NO: 1017 - RNA, 21 nt, Artificial sequence
  F12 RNAi agent sense strand modified sequence
ggaacccggacaacgacaauu

SEQ ID NO: 1018 - RNA, 21 nt, Artificial sequence
  F12 RNAi agent sense strand modified sequence
cgcaagagucugucuucgauu

SEQ ID NO: 1019 - RNA, 21 nt, Artificial sequence
  F12 RNAi agent sense strand modified sequence
cgcaagagucugucuucgauu

SEQ ID NO: 1020 - RNA, 21 nt, Artificial sequence
  F12 RNAi agent sense strand modified sequence
cgcaagagucugucuucgauu

SEQ ID NO: 1021 - RNA, 21 nt, Artificial sequence
  F12 RNAi agent sense strand modified sequence
cgcaagagucugucuucgauu

SEQ ID NO: 1022 - RNA, 21 nt, Artificial sequence
  F12 RNAi agent sense strand modified sequence
cgcuccugucgccuuacguuu

SEQ ID NO: 1023 - RNA, 21 nt, Artificial sequence
  F12 RNAi agent sense strand modified sequence
cgcuccugucgccuuacgauu

SEQ ID NO: 1024 - RNA, 21 nt, Artificial sequence
  F12 RNAi agent sense strand modified sequence
cgcuccugucgccuuacgauu

SEQ ID NO: 1025 - RNA, 21 nt, Artificial sequence
  F12 RNAi agent sense strand modified sequence
cgcuccugucgccuuacgauu

SEQ ID NO: 1026 - RNA, 21 nt, Artificial sequence
  F12 RNAi agent sense strand modified sequence
cgcuccugucgccuuacgauu

SEQ ID NO: 1027 - RNA, 21 nt, Artificial sequence
  F12 RNAi agent sense strand base sequence
aacucaauaaagugcugugaa